European Patent Application EP 4 112 073 A1, published January 4, 2023. Title: Recombinant HVT Vectors Expressing Antigens of Avian Pathogens and Uses Thereof. Applicant: Boehringer Ingelheim Animal Health USA Inc. The sequence listing filed with the application follows.

SEQUENCE LISTING (47 sequences)

SEQ ID NO: 1 - DNA, 1665 bp, artificial sequence
  NDV-F VIId codon-optimized DNA sequence
atgggcagcaagcccagcacaagaatcccagcccccctgatgctgatcacccgcatcatgctgatcctgggctgcatcagacccacaagctccctggatggacgccccctggccgctgccggcatcgtggtgaccggcgacaaggccgtgaacgtgtacaccagcagccagaccggcagcatcatcgtgaagctgctgcccaacatgcccagagacaaagaggcctgcgccaaggcccccctggaagcctacaacagaaccctgaccaccctgctgacccccctgggcgacagcatcagaaagatccagggctccgtgagcacaagcggcggaggaaagcagggcagactgatcggcgccgtgatcggcagcgtggccctgggagtggctacagctgcccagattaccgctgcagccgccctgatccaggccaaccagaacgccgccaacatcctgagactgaaagagagcattgccgccaccaacgaggccgtgcacgaagtgaccgacggcctgagccagctgtccgtggccgtgggcaagatgcagcagttcgtgaacgaccagttcaacaacaccgccagagagctggactgcatcaagatcacccagcaggtgggcgtggagctgaacctgtacctgaccgagctgaccacagtgttcggcccccagatcacaagcccagccctgacacagctgaccatccaggccctgtacaacctggctggcggcaacatggactatctgctgacaaagctgggaatcggcaacaaccagctgtccagcctgatcggaagcggcctgatcaccggctaccccatcctgtacgacagccagacacagctgctgggcatccaggtgaacctgcccagcgtgggcaacctgaacaacatgcgcgccacctacctggaaaccctgagcgtgtccaccaccaagggctacgccagcgccctggtgcccaaggtggtgacacaggtgggcagcgtgatcgaggaactggacaccagctactgcatcgagagcgacctggacctgtactgcaccagaatcgtgaccttcccaatgagccccggcatctacagctgcctgagcggcaacaccagcgcctgcatgtacagcaagaccgaaggcgcactgacaacaccctacatggccctgaagggaagcgtgatcgccaactgcaagatcaccacctgcagatgcaccgaccccccaggcatcatcagccagaactacggcgaggccgtgagcctgatcgatcgccattcctgtaacgtgctgtccctggacggcatcacactgagactgagcggcgagttcgatgccacctaccagaagaacatcagcatcctggacagccaggtgatcgtgaccggcaacctggacatcagcaccgagctgggcaacgtgaataacagcatcagcaacgccctggacagactggccgagagcaacagcaagctggaaaaagtgaacgtgcgcctgacatccacttccgctctgatcacctacatcgtgctgaccgtgatcagcctggtgttcggcgccctgagcctggtgctggcctgctacctgatgtacaagcagaaggcccagcagaaaaccctgctgtggctgggcaacaacaccctggaccagatgagagccaccaccagagcctgatga

SEQ ID NO: 2 - protein, 553 aa, artificial sequence
  NDV-F protein sequence from codon-optimized VIId gene
MGSKPSTRIPAPLMLITRIMLILGCIRPTSSLDGRPLAAAGIVVTGDKAVNVYTSSQTGSIIVKLLPNMPRDKEACAKAPLEAYNRTLTTLLTPLGDSIRKIQGSVSTSGGGKQGRLIGAVIGSVALGVATAAQITAAAALIQANQNAANILRLKESIAATNEAVHEVTDGLSQLSVAVGKMQQFVNDQFNNTARELDCIKITQQVGVELNLYLTELTTVFGPQITSPALTQLTIQALYNLAGGNMDYLLTKLGIGNNQLSSLIGSGLITGYPILYDSQTQLLGIQVNLPSVGNLNNMRATYLETLSVSTTKGYASALVPKVVTQVGSVIEELDTSYCIESDLDLYCTRIVTFPMSPGIYSCLSGNTSACMYSKTEGALTTPYMALKGSVIANCKITTCRCTDPPGIISQNYGEAVSLIDRHSCNVLSLDGITLRLSGEFDATYQKNISILDSQVIVTGNLDISTELGNVNNSISNALDRLAESNSKLEKVNVRLTSTSALITYIVLTVISLVFGALSLVLACYLMYKQKAQQKTLLWLGNNTLDQMRATTRA

SEQ ID NO: 3 - DNA, 1662 bp, artificial sequence
  NDV-F VIId wildtype DNA sequence
atgggctccaaaccttctaccaggatcccagcacctctgatgctgatcacccggattatgctgatattgggctgtatccgtccgacaagctctcttgacggcaggcctcttgcagctgcaggaattgtagtaacaggagataaggcagtcaatgtatacacttcgtctcagacagggtcaatcatagtcaagttgctcccgaatatgcccagggataaggaggcgtgtgcaaaagccccattagaggcatataacagaacactgactactttgctcactcctcttggcgactccatccgcaagatccaagggtctgtgtccacatctggaggaggcaagcaaggccgcctgataggtgctgttattggcagtgtagctcttggggttgcaacagcggcacagataacagcagctgcggccctaatacaagccaaccagaatgccgccaacatcctccggcttaaggagagcattgctgcaaccaatgaagctgtgcatgaagtcaccgacggattatcacaactatcagtggcagttgggaagatgcagcagtttgtcaatgaccagtttaataatacggcgcgagaattggactgtataaaaatcacacaacaggttggtgtagaactcaacctatacctaactgaattgactacagtattcgggccacagatcacctcccctgcattaactcagctgaccatccaggcactttataatttagctggtggcaatatggattacttattaactaagttaggtatagggaacaatcaactcagctcgttaattggtagcggcctgatcactggttaccctatactgtatgactcacagactcaactcttgggcatacaagtgaatttaccctcagtcgggaacttaaataatatgcgtgccacctatttggagaccttatctgtaagtacaaccaaaggatatgcctcagcacttgtcccgaaagtagtgacacaagtcggttccgtgatagaagagcttgacacctcatactgtatagagtccgatctggatttatattgtactagaatagtgacattccccatgtccccaggtatttattcctgtttgagcggcaacacatcagcttgcatgtattcaaagactgaaggcgcactcactacgccgtatatggcccttaaaggctcagttattgccaattgtaaaataacaacatgtagatgtacagaccctcctggtatcatatcgcaaaattatggagaagctgtatccctgatagatagacattcgtgcaatgtcttatcattagacgggataactctaaggctcagtggggaatttgatgcaacttatcaaaagaacatctcaatactagattctcaagtcatcgtgacaggcaatcttgatatatcaactgaacttggaaacgtcaacaattcaatcagcaatgccttggataggttggcagaaagcaacagcaagctagaaaaagtcaatgtcagactaaccagcacatctgctctcattacctatattgttctaactgtcatttctctagttttcggtgcacttagtctggtgttagcgtgttacctgatgtacaaacagaaggcacaacaaaagaccttgctatggcttgggaataataccctcgatcagatgagagccactacaagagcatga

SEQ ID NO: 4 - protein, 553 aa, artificial sequence; identical to SEQ ID NO: 2
  NDV-F protein from wildtype VIId DNA sequence

SEQ ID NO: 5 - DNA, 1665 bp, artificial sequence
  NDV-F Ca02 codon-optimized DNA sequence
atgggcagcaagcccagcacctggatcagcgtgaccctgatgctgatcaccagaaccatgctgatcctgagctgcatctgccccacaagcagcctggacggcagacccctggccgctgccggcatcgtggtgaccggcgacaaggccgtgaacatctacaccagcagccagaccggcagcatcatcatcaagctgctgcccaacatgcccaaggacaaagaggcctgcgccaaggcccccctggaagcctacaacagaaccctgaccaccctgctgacccccctgggcgacagcatcagaagaatccagggcagcgccaccacaagcggcggaggaaagcagggcagactggtgggcgctatcatcgggagcgtggccctgggcgtggccacagctgcccagattaccgctgcagccgccctgattcaggccaatcagaacgccgccaacatcctgagactgaaagagagcattgccgccaccaacgacgccgtgcacgaagtgacaaacggactgtcccagctggctgtcgctgtcggcaagatgcagcagttcgtgaacaaccagttcaacaacaccgccagagagctggactgcatcaagatcgcccagcaggtgggcgtggagctgaacctgtacctgaccgagctgaccacagtgttcggcccccagatcacaagccccgctctgacccagctgacaatccaggccctgtacaacctggctggcggcaacatggactatctgctgactaagctgggagtgggcaacaaccagctgtccagcctgatcgggtccgggctgatcacaggcaaccccatcctgtacgacagccagacacagctgctgggcatccagatcaacctgccatccgtgggaagcctgaacaacatgagagccacctacctggaaaccctgagcgtgtccaccaccaagggcttcgccagcgccctggtgcccaaggtggtgacacaggtgggcagcgtgatcgaggaactggacaccagctactgcatcgagagcgacatcgacctgtactgcaccagagtggtgaccttcccaatgagccccggcatctacagctgcctgagcggcaacaccagcgcctgcatgtacagcaagaccgaaggagcactgacaacaccctacatggccctgaagggaagcgtgatcgccaactgcaagatgaccacctgcagatgcgccgaccccccaggcatcatcagccagaactacggcgaggccgtgagcctgatcgacaaacattcctgtagcgtgctgtccctggatggcatcacactgagactgagcggcgagttcgacgccacctaccagaagaacatcagcatcctggacagccaggtgatcgtgaccggcaacctggacatcagcaccgagctgggcaacgtgaacaacagcatcagcagcaccctggacaagctggccgagtccaacaacaagctgaacaaagtgaacgtgaacctgaccagcacaagcgccctgatcacctacatcgtgctggccatcgtgtccctggccttcggcgtgatcagcctggtgctggcctgctacctgatgtacaagcagagagcccagcagaaaaccctgctgtggctgggcaataacaccctggaccagatgagggccaccaccagaacctgatga

SEQ ID NO: 6 - protein, 553 aa, artificial sequence
  NDV-F protein sequence from codon-optimized CA02 gene
MGSKPSTWISVTLMLITRTMLILSCICPTSSLDGRPLAAAGIVVTGDKAVNIYTSSQTGSIIIKLLPNMPKDKEACAKAPLEAYNRTLTTLLTPLGDSIRRIQGSATTSGGGKQGRLVGAIIGSVALGVATAAQITAAAALIQANQNAANILRLKESIAATNDAVHEVTNGLSQLAVAVGKMQQFVNNQFNNTARELDCIKIAQQVGVELNLYLTELTTVFGPQITSPALTQLTIQALYNLAGGNMDYLLTKLGVGNNQLSSLIGSGLITGNPILYDSQTQLLGIQINLPSVGSLNNMRATYLETLSVSTTKGFASALVPKVVTQVGSVIEELDTSYCIESDIDLYCTRVVTFPMSPGIYSCLSGNTSACMYSKTEGALTTPYMALKGSVIANCKMTTCRCADPPGIISQNYGEAVSLIDKHSCSVLSLDGITLRLSGEFDATYQKNISILDSQVIVTGNLDISTELGNVNNSISSTLDKLAESNNKLNKVNVNLTSTSALITYIVLAIVSLAFGVISLVLACYLMYKQRAQQKTLLWLGNNTLDQMRATTRT

SEQ ID NO: 7 - DNA, 1362 bp, artificial sequence
  IBDV DNA sequence encoding VP2
atgacaaacctgcaagatcaaacccaacagattgttccgttcatacggagccttctgatgccaacaaccggaccggcgtccattccggacgacaccctggagaagcacactctcaggtcagagacctcgacctacaatttgactgtgggggacacagggtcagggctaattgtctttttccctggattccctggctcaattgtgggtgctcactacacactgcagagcaatgggaactacaagttcgatcagatgctcctgactgcccagaacctaccggccagctacaactactgcagactagtgagtcggagtctcacagtgaggtcaagcacactccctggtggcgtttatgcactaaacggcaccataaacgccgtgaccttccaaggaagcctgagtgaactgacagatgttagctacaatgggttgatgtctgcaacagccaacatcaacgacaaaattgggaatgtcctggtaggggaaggggtcactgtcctcagcctacccacatcatatgatcttgggtatgtgaggcttggtgaccccattcccgctatagggcttgacccaaaaatggtagctacatgcgacagcagtgacaggcccagagtctacaccataactgcagccgatgattaccaattctcatcacagtaccaaccaggtggggtaacaatcacactgttctcagccaacattgatgctatcacaagcctcagcattgggggagagctcgtgtttcaaacaagcgtccaaggccttgtactgggcgccaccatctaccttataggctttgatgggactgcggtaatcaccagagctgtagccgcagataatgggctgacggccggcaccgacaatcttatgccattcaatcttgtcattccaaccaatgagataacccagccaatcacatccatcaaactggagatagtgacctccaaaagtggtggtcaggcaggggatcagatgtcatggtcggcaagtgggagcctagcagtgacgatccatggtggcaactatccaggggccctccgtcccgtcacactagtagcctacgaaagagtggcaacaggatccgtcgttacggtcgctggggtgagtaacttcgagctgattccaaatcctgaactagcaaagaacctggttacagaatacggccgatttgacccaggagccatgaactacacaaaattgatactgagtgagagggaccgtcttggcatcaagaccgtctggccaacaagggagtacactgattttcgtgagtacttcatggaggtggccgacctcaactctcccctgaagattgcaggagcatttggcttcaaagacataatccgggctataaggaggtaa

SEQ ID NO: 8 - protein, 453 aa, artificial sequence
  IBDV VP2 protein
MTNLQDQTQQIVPFIRSLLMPTTGPASIPDDTLEKHTLRSETSTYNLTVGDTGSGLIVFFPGFPGSIVGAHYTLQSNGNYKFDQMLLTAQNLPASYNYCRLVSRSLTVRSSTLPGGVYALNGTINAVTFQGSLSELTDVSYNGLMSATANINDKIGNVLVGEGVTVLSLPTSYDLGYVRLGDPIPAIGLDPKMVATCDSSDRPRVYTITAADDYQFSSQYQPGGVTITLFSANIDAITSLSIGGELVFQTSVQGLVLGATIYLIGFDGTAVITRAVAADNGLTAGTDNLMPFNLVIPTNEITQPITSIKLEIVTSKSGGQAGDQMSWSASGSLAVTIHGGNYPGALRPVTLVAYERVATGSVVTVAGVSNFELIPNPELAKNLVTEYGRFDPGAMNYTKLILSERDRLGIKTVWPTREYTDFREYFMEVADLNSPLKIAGAFGFKDIIRAIRR

SEQ ID NO: 9 - DNA, 368 bp, artificial sequence
  SV40 promoter
gaattcgagctcggtacagcttggctgtggaatgtgtgtcagttagggtgtggaaagtccccaggctccccagcaggcagaagtatgcaaagcatgcatctcaattagtcagcaaccaggtgtggaaagtccccaggctccccagcaggcagaagtatgcaaagcatgcatctcaattagtcagcaaccatagtcccgcccctaactccgcccatcccgcccctaactccgcccagttccgcccattctccgccccatggctgactaattttttttatttatgcagaggccgaggccgcctcggcctctgagctattccagaagtagtgaggaggcttttttggaggcctaggcttttgcaaaaagct

SEQ ID NO: 10 - DNA, 1391 bp, artificial sequence
  CMV-IE promoter
aactccgcccgttttatgactagaaccaatagtttttaatgccaaatgcactgaaatcccctaatttgcaaagccaaacgccccctatgtgagtaatacggggactttttacccaatttcccaagcggaaagccccctaatacactcatatggcatatgaatcagcacggtcatgcactctaatggcggcccatagggactttccacatagggggcgttcaccatttcccagcataggggtggtgactcaatggcctttacccaagtacattgggtcaatgggaggtaagccaatgggtttttcccattactggcaagcacactgagtcaaatgggactttccactgggttttgcccaagtacattgggtcaatgggaggtgagccaatgggaaaaacccattgctgccaagtacactgactcaatagggactttccaatgggtttttccattgttggcaagcatataaggtcaatgtgggtgagtcaatagggactttccattgtattctgcccagtacataaggtcaatagggggtgaatcaacaggaaagtcccattggagccaagtacactgcgtcaatagggactttccattgggttttgcccagtacataaggtcaataggggatgagtcaatgggaaaaacccattggagccaagtacactgactcaatagggactttccattgggttttgcccagtacataaggtcaatagggggtgagtcaacaggaaagtcccattggagccaagtacattgagtcaatagggactttccaatgggttttgcccagtacataaggtcaatgggaggtaagccaatgggtttttcccattactggcacgtatactgagtcattagggactttccaatgggttttgcccagtacataaggtcaataggggtgaatcaacaggaaagtcccattggagccaagtacactgagtcaatagggactttccattgggttttgcccagtacaaaaggtcaatagggggtgagtcaatgggtttttcccattattggcacgtacataaggtcaataggggtgagtcattgggtttttccagccaatttaattaaaacgccatgtactttcccaccattgacgtcaatgggctattgaaactaatgcaacgtgacctttaaacggtactttcccatagctgattaatgggaaagtaccgttctcgagccaatacacgtcaatgggaagtgaaagggcagccaaaacgtaacaccgccccggttttcccctggaaattccatattggcacgcattctattggctgagctgcgttctacgtgggtataagaggcgcgaccagcgtcggtaccgtcgcagtcttcggtctgaccaccgtagaacgcagagctcctcgctgcag

SEQ ID NO: 11 - DNA, 218 bp, artificial sequence
  SV40 polyA signal
ggggatccagacatgataagatacattgatgagtttggacaaaccacaactagaatgcagtgaaaaaaatgctttatttgtgaaatttgtgatgctattgctttatttgtaaccattataagctgcaataaacaagttaacaacaacaattgcattgattttatgtttcaggttcagggggaggtgtgggaggttttttcggatcctctagagtcgac

SEQ ID NO: 12 - DNA, 155 bp, artificial sequence
  Synthetic polyA signal
aataaaatatctttattttcattacatctgtgtgttggttttttgtgtgaatcgatagtactaacatacgctctccatcaaaacaaaacgaaacaaaacaaactagcaaaataggctgtccccagtgcaagtgcaggtgccagaacatttctctt

SEQ ID NO: 13 - DNA, 22 bp, artificial sequence
  primer
cgaacaaacttcatcgctatgc

SEQ ID NO: 14 - DNA, 22 bp, artificial sequence
  primer
taactcaaatgcgaagcgttgc

SEQ ID NO: 15 - DNA, 21 bp, artificial sequence
  primer
actgacaacaccctacatggc

SEQ ID NO: 16 - DNA, 19 bp, artificial sequence
  VIioptF RP primer
gccagcaccaggctcaggg

SEQ ID NO: 17 - DNA, 18 bp, artificial sequence
  primer
agcttggctgtggaatgt

SEQ ID NO: 18 - DNA, 4344 bp, artificial sequence
  Partial plasmid pHM103+Fopt DNA sequence
gagctcagggtatgatactcagctgttattgtggccgaccaggaggactccaatgcttagcattcataagaacgctagagatgctatttaacgatgtgctgtcgtctaaagaatttgtgcatttagcctttaaatgtaaaaccaatgacgcattcactacgctcgtgcgtgcaatttctgggccagggtatgcatattccataacagaaatcgacacttgagaagaggatctgactgtttgggataaaggtcgtttgggtctgtcctagcgatataatttatatgacgatatacattaaacatctgtgtgcagtacttaggtatttaatcatgtcgatgaaatgttatgtgtaaatatcggacaatatagataacgggcacgctgctattgtaacgtgcgcccgcgcgctagtgctgactaatagtgtggatgatgtatacagtatattacaaacggaaatgatacgtaataaattatgtactcttattgatttataaaaacatacatgcagtgttgctatgtcacataattagcctcgcccgtctacgctccactgaagataatgggctcccgctgttcaaaaaaatcagcgtgcgtcgataagactttggtgcagtctcttcggggtcgcaatttagatttgccgcatggagggtatctggggatttttgccaatgctggagcgacgactgtacgattcgtcccatcgggatctagcagaccaatgatgttgacacacatcggccatgcatgtacggacggtctattgcgcgagtttgttattttcgaaggacaagatggaagtgtatatggaaccgacaataatgttagtttgcatttcttagggcggaatctacatgatatcttatccaagcggggtatgagccagagagatgtgatggtcataaagggtaaattttttagatctgaaataacgcagttgcccaaacaacgatcgcgattaaaagaaaaatcggatggttcaattaggacatgcatggattctgtgcgcataaaccataaccgcagcactgttgggcacttcggtaactcaaatgcgaagcgttgcacgtctgcgataactacgcctactatgcacattgttactcctgcatcttaaaaatatatcctgtagtaattttcacagcaatgtcataacatcatctcgctaaagaatgacctgggattggagaagtaatgaatatttgcaaccaatgcattgaataaactaacattaaacgaattcgagctcggtacagcttggctgtggaatgtgtgtcagttagggtgtggaaagtccccaggctccccagcaggcagaagtatgcaaagcatgcatctcaattagtcagcaaccaggtgtggaaagtccccaggctccccagcaggcagaagtatgcaaagcatgcatctcaattagtcagcaaccatagtcccgcccctaactccgcccatcccgcccctaactccgcccagttccgcccattctccgccccatggctgactaattttttttatttatgcagaggccgaggccgcctcggcctctgagctattccagaagtagtgaggaggcttttttggaggcctaggcttttgcaaaaagctgcggccgccaccatgggcagcaagcccagcacaagaatcccagcccccctgatgctgatcacccgcatcatgctgatcctgggctgcatcagacccacaagctccctggatggacgccccctggccgctgccggcatcgtggtgaccggcgacaaggccgtgaacgtgtacaccagcagccagaccggcagcatcatcgtgaagctgctgcccaacatgcccagagacaaagaggcctgcgccaaggcccccctggaagcctacaacagaaccctgaccaccctgctgacccccctgggcgacagcatcagaaagatccagggctccgtgagcacaagcggcggaggaaagcagggcagactgatcggcgccgtgatcggcagcgtggccctgggagtggctacagctgcccagattaccgctgcagccgccctgatccaggccaaccagaacgccgccaacatcctgagactgaaagagagcattgccgccaccaacgaggccgtgcacgaagtgaccgacggcctgagccagctgtccgtggccgtgggcaagatgcagcagttcgtgaacgaccagttcaacaacaccgccagagagctggactgcatcaagatcacccagcaggtgggcgtggagctgaacctgtacctgaccgagctgaccacagtgttcggcccccagatcacaagcccagccctgacacagctgaccatccaggccctgtacaacctggctggcggcaacatggactatctgctgacaaagctgggaatcggcaacaaccagctgtccagcctgatcggaagcggcctgatcaccggctaccccatcctgtacgacagccagacacagctgctgggcatccaggtgaacctgcccagcgtgggcaacctgaacaacatgcgcgccacctacctggaaaccctgagcgtgtccaccaccaagggctacgccagcgccctggtgcccaaggtggtgacacaggtgggcagcgtgatcgaggaactggacaccagctactgcatcgagagcgacctggacctgtactgcaccagaatcgtgaccttcccaatgagccccggcatctacagctgcctgagcggcaacaccagcgcctgcatgtacagcaagaccgaaggcgcactgacaacaccctacatggccctgaagggaagcgtgatcgccaactgcaagatcaccacctgcagatgcaccgaccccccaggcatcatcagccagaactacggcgaggccgtgagcctgatcgatcgccattcctgtaacgtgctgtccctggacggcatcacactgagactgagcggcgagttcgatgccacctaccagaagaacatcagcatcctggacagccaggtgatcgtgaccggcaacctggacatcagcaccgagctgggcaacgtgaataacagcatcagcaacgccctggacagactggccgagagcaacagcaagctggaaaaagtgaacgtgcgcctgacatccacttccgctctgatcacctacatcgtgctgaccgtgatcagcctggtgttcggcgccctgagcctggtgctggcctgctacctgatgtacaagcagaaggcccagcagaaaaccctgctgtggctgggcaacaacaccctggaccagatgagagccaccaccagagcctgatgagcggccgcggggatccagacatgataagatacattgatgagtttggacaaaccacaactagaatgcagtgaaaaaaatgctttatttgtgaaatttgtgatgctattgctttatttgtaaccattataagctgcaataaacaagttaacaacaacaattgcattgattttatgtttcaggttcagggggaggtgtgggaggttttttcggatcctctagagtcgacaattattttatttaataacatatagcccaaagacctctatgaacatttagtttcccgtatactcaacggcgcgtgtacacacgcatctctttgcatagcgatgaagtttgttcggcagcagaaaatgcagatatccaacaatctggagaaaacttatcatcacagtggcagtggaaacataccccctctatattcatggtataattatcgtctacagcgtccaggatagtggcgtgagaaaatggagatctgcagccctcctttccatggcatgccgctttattgttcattaaacgcacaatggtctcaacgccagatatgggcatagattctgaagaacccgttgacaatccgaagaagaaggcgtgcaggtctttggaagactcgcacgttggtcttataatgtatgatcgagatgtcaccctaatgccacatggtacaggcttatcgcggtcatggcgatcggacttgtaatttgcaacgatgggcaaaggatcgacgacatgccaaacattctgaacccgtagagatgttaacgatgacgaggatgaatatcccatgctcgctgccatagtatcaagtacaccgcgaataaggacgcgtccaacatcgttatatgcacacaatgggctacacgtgactaacacccccgaatattagtcatatgtgagtttcagtctggctcccatatagcctgtagactatttgtggtttaagtgtgaacgaggcgctgtgaacgagactcgggccgattgtaagaacaagcaaatgcactttccatttaacaagaagtgtagagagaatactcaacctctttggatgtatcctcgag

SEQ ID NO: 19 - DNA, 4085 bp, artificial sequence
  Partial plasmid pSB1 44cds SV FCAopt sequence for vSB1-009
cttttgtcatgctcggagctctgatcgcatcttatcattacgtctgcatagcaacgtctggagacgtgacgtggaagaccgggtttttagttgtggcggcagggacgattgccggcatcacggctccgtatggagacatttctcctctagccggctttctttcggcgtatacggcgttagctattcacgtggtcagagacgccagtcggtctctaatgaacacgtgctactaccgtgcacgtcgggaaattactgtgaacggtgcatatcgcctcggtcgcgcgcgtctcccgcccagcacggacgccgaggcgacgcgcgaagaagacgtatccagttacgatacgctgggggggaatattcctacgataattctgagcctcatagcggtcatctcgattccagccatagccagctttcaaaagtacatgtcgaacgcaactaagcaccagtcaacattgactgacacgttacgcagtatatgcggtttcttggtgggtacaagtgtcgcgatattccttccgtcgcgctaccacgaggttctgttccgtccaattcttgtattactgttaatattcggggcaatggctactaccttagccggcttcggtttacttctcgggccgacattgttttccgcgacagccgcggttctgtgctgctacacttgtataaatgtacgcaacgcgaatagcggaataaagcaattggcggccgccgcagctggtaaatgcatattaggaactgccatctcgagcatgttggtttgcgtgttaatacaatattcctgatcgcggagcgattaatttttatatcatgtgctcatagcgttctttcgaactgcgaataaaactttcgtggctactaaaggggcctatcgtgggtttatgcgctgtcgaaaacatgaaagggccgatttaaagctaagttgcgcaggcagaggccactccatatacgctctcggagacgcggctcgcacgccagctgaaatattttcccccctgcaggtcgacccaattcgagctcggtacagcttggctgtggaatgtgtgtcagttagggtgtggaaagtccccaggctccccagcaggcagaagtatgcaaagcatgcatctcaattagtcagcaaccaggtgtggaaagtccccaggctccccagcaggcagaagtatgcaaagcatgcatctcaattagtcagcaaccatagtcccgcccctaactccgcccatcccgcccctaactccgcccagttccgcccattctccgccccatggctgactaattttttttatttatgcagaggccgaggccgcctcggcctctgagctattccagaagtagtgaggaggcttttttggaggcctaggcttttgcaaaaagctcccggggcggccgccaccatgggcagcaagcccagcacctggatcagcgtgaccctgatgctgatcaccagaaccatgctgatcctgagctgcatctgccccacaagcagcctggacggcagacccctggccgctgccggcatcgtggtgaccggcgacaaggccgtgaacatctacaccagcagccagaccggcagcatcatcatcaagctgctgcccaacatgcccaaggacaaagaggcctgcgccaaggcccccctggaagcctacaacagaaccctgaccaccctgctgacccccctgggcgacagcatcagaagaatccagggcagcgccaccacaagcggcggaggaaagcagggcagactggtgggcgctatcatcgggagcgtggccctgggcgtggccacagctgcccagattaccgctgcagccgccctgattcaggccaatcagaacgccgccaacatcctgagactgaaagagagcattgccgccaccaacgacgccgtgcacgaagtgacaaacggactgtcccagctggctgtcgctgtcggcaagatgcagcagttcgtgaacaaccagttcaacaacaccgccagagagctggactgcatcaagatcgcccagcaggtgggcgtggagctgaacctgtacctgaccgagctgaccacagtgttcggcccccagatcacaagccccgctctgacccagctgacaatccaggccctgtacaacctggctggcggcaacatggactatctgctgactaagctgggagtgggcaacaaccagctgtccagcctgatcgggtccgggctgatcacaggcaaccccatcctgtacgacagccagacacagctgctgggcatccagatcaacctgccatccgtgggaagcctgaacaacatgagagccacctacctggaaaccctgagcgtgtccaccaccaagggcttcgccagcgccctggtgcccaaggtggtgacacaggtgggcagcgtgatcgaggaactggacaccagctactgcatcgagagcgacatcgacctgtactgcaccagagtggtgaccttcccaatgagccccggcatctacagctgcctgagcggcaacaccagcgcctgcatgtacagcaagaccgaaggagcactgacaacaccctacatggccctgaagggaagcgtgatcgccaactgcaagatgaccacctgcagatgcgccgaccccccaggcatcatcagccagaactacggcgaggccgtgagcctgatcgacaaacattcctgtagcgtgctgtccctggatggcatcacactgagactgagcggcgagttcgacgccacctaccagaagaacatcagcatcctggacagccaggtgatcgtgaccggcaacctggacatcagcaccgagctgggcaacgtgaacaacagcatcagcagcaccctggacaagctggccgagtccaacaacaagctgaacaaagtgaacgtgaacctgaccagcacaagcgccctgatcacctacatcgtgctggccatcgtgtccctggccttcggcgtgatcagcctggtgctggcctgctacctgatgtacaagcagagagcccagcagaaaaccctgctgtggctgggcaataacaccctggaccagatgagggccaccaccagaacctgatgagcggccgcgatacctgcaggtttgcggtgacattgatctggctcattatatgccccgagctcttgtaacatcgcggacgcgatttccgtagtaggcacatctcaaatgcaaaagcggcatgtcaaccgtataggtacatccggccctgcttacagtcggtagggcatatatccaccggaaaacttcagctttagactcctcaggtgatgaggaatagtatgtaaccctctagcagtacggtatttctaaaaaaaggtagatccttttccacacggcacagactaaataacgtacactacacaggttctctcgaacttcgtttggaccggaattattccctcggcagcgcctaaaaagcaaacctctagagtagataagtgtcagtgaacctaggccttctttgttccacggctggaaagctaagggacgaggtacacgcgaccccagccacgcacgaacagagtttaacggaagcgtcgtttgcgggataaggttgtcggaccccgcgggtccgttgaaaagtggctgcgcgcctaccgacgaatacgtcggtaacaattttagaaatcgaatatgactgcgagtaccgtacaatcgcgaaatacggtctctatatagctactcggtccttaaatatgtaagtatgatgtcccctactcccgaagacgaccgcgacttggtcgcagtacgtgggctgctccggatgatggacgagaccacatctgagcgacacaaacgttcgcgttcaggatgcccccggttgttatgcggttgtacgatcgggatcgctcttactgtgttcgtcatcacagctacggtcgtgctagcttcgctgtttgcattctcttacatgtccctggagtccggtacatgtcctcacgaatggatcggtttaggctatagttgtatgcgcgcgatggggagcaacgctaccgagctagaagccctagatacgtgctcccgacataacagcaagcttgtcgactttactcatgcgaaaattctaatcgaagctatcgc

SEQ ID NO: 20 - DNA, 4335 bp, artificial sequence
  Partial plasmid pHVT US2 SV-Fopt-SynPA for vHVT306
taaaatgggatctatcattacattcgttaagagtctggataattttactgtttgccagcttcgatcttggaacgtactgtggatagtgccttacttggaatcgtgaaaatttgaaacgtccattatttggatatcttccggttgtcccatatcccgccctggtaccgctcggataccttgcccgtatggattcgtattgacagtcgcgcaatcggggaccaacaacgcgtgggtccacactcattcggaaattttccgatgattctgaatatttattgccgctcgttacgagtcgttggacatatctgtaatacatttcttcttctgaaggatcgctgcacatttgatctatacattggccaggatgttcaagtctcagatgttgcattctggcacagcacaactttatggcatttccgatgtaatcgtccggcagccctgggggagttctatattcgcatattgggatggtaaggacaatagcagatctcgcaacctccagggaggctataataacgtttttaaaggatggatttctcataaaaatctgtcgcaaattacactgagaatatcctttactagcgccgattgagagcatcgtcgtccaattttctaaatggaaagaaaacaaggcgggcaagagtgttccaaacattttcattttcggcgaatctctcaaatcccatggcgtgcaattgattgcaaaattggcacttccgttcacgtttgtatctccaaactctaagacacttttaattgaaaaactacgttctagtgtggaaagaaacctataggcagaccatagaactatttgacaccacatatctttttgtatgtcaaactgaccatgatcgtatgttgctgaatgcactagggcaattcgctcgcgcgactccatacattgaataattccacacgtcagctcatcggttagcaaggtccagtagttgaagtcatttatttttccccgcggctggccaaatctacctctgggaatatccaagttgtcgaatatgatcgcaccggctctggtcatggtgaaggaacttgtagcataaagacgcaggtatcataggggtaatatttttttattcactcacatactaaaagtaacgcatattagcaccatgtatgggctatcaattgacatttgcgtagcactacatcacgattatgtacaacataatgggacaacatatgcctgcaggtcgacccaattcgagctcggtacagcttggctgtggaatgtgtgtcagttagggtgtggaaagtccccaggctccccagcaggcagaagtatgcaaagcatgcatctcaattagtcagcaaccaggtgtggaaagtccccaggctccccagcaggcagaagtatgcaaagcatgcatctcaattagtcagcaaccatagtcccgcccctaactccgcccatcccgcccctaactccgcccagttccgcccattctccgccccatggctgactaattttttttatttatgcagaggccgaggccgcctcggcctctgagctattccagaagtagtgaggaggcttttttggaggcctaggcttttgcaaaaagctcccggggcggccgccaccatgggcagcaagcccagcacaagaatcccagcccccctgatgctgatcacccgcatcatgctgatcctgggctgcatcagacccacaagctccctggatggacgccccctggccgctgccggcatcgtggtgaccggcgacaaggccgtgaacgtgtacaccagcagccagaccggcagcatcatcgtgaagctgctgcccaacatgcccagagacaaagaggcctgcgccaaggcccccctggaagcctacaacagaaccctgaccaccctgctgacccccctgggcgacagcatcagaaagatccagggctccgtgagcacaagcggcggaggaaagcagggcagactgatcggcgccgtgatcggcagcgtggccctgggagtggctacagctgcccagattaccgctgcagccgccctgatccaggccaaccagaacgccgccaacatcctgagactgaaagagagcattgccgccaccaacgaggccgtgcacgaagtgaccgacggcctgagccagctgtccgtggccgtgggcaagatgcagcagttcgtgaacgaccagttcaacaacaccgccagagagctggactgcatcaagatcacccagcaggtgggcgtggagctgaacctgtacctgaccgagctgaccacagtgttcggcccccagatcacaagcccagccctgacacagctgaccatccaggccctgtacaacctggctggcggcaacatggactatctgctgacaaagctgggaatcggcaacaaccagctgtccagcctgatcggaagcggcctgatcaccggctaccccatcctgtacgacagccagacacagctgctgggcatccaggtgaacctgcccagcgtgggcaacctgaacaacatgcgcgccacctacctggaaaccctgagcgtgtccaccaccaagggctacgccagcgccctggtgcccaaggtggtgacacaggtgggcagcgtgatcgaggaactggacaccagctactgcatcgagagcgacctggacctgtactgcaccagaatcgtgaccttcccaatgagccccggcatctacagctgcctgagcggcaacaccagcgcctgcatgtacagcaagaccgaaggcgcactgacaacaccctacatggccctgaagggaagcgtgatcgccaactgcaagatcaccacctgcagatgcaccgaccccccaggcatcatcagccagaactacggcgaggccgtgagcctgatcgatcgccattcctgtaacgtgctgtccctggacggcatcacactgagactgagcggcgagttcgatgccacctaccagaagaacatcagcatcctggacagccaggtgatcgtgaccggcaacctggacatcagcaccgagctgggcaacgtgaataacagcatcagcaacgccctggacagactggccgagagcaacagcaagctggaaaaagtgaacgtgcgcctgacatccacttccgctctgatcacctacatcgtgctgaccgtgatcagcctggtgttcggcgccctgagcctggtgctggcctgctacctgatgtacaagcagaaggcccagcagaaaaccctgctgtggctgggcaacaacaccctggaccagatgagagccaccaccagagcctgatgagcggccgcgatatcaataaaatatctttattttcattacatctgtgtgttggttttttgtgtgaatcgatagtactaacatacgctctccatcaaaacaaaacgaaacaaaacaaactagcaaaataggctgtccccagtgcaagtgcaggtgccagaacatttctcttctagacctgcaggcccgggcaagtagatgcaatttcctcacactagttgggtttatctactattgaattttcccctatctgtgatacacttgggagcctctacaagcatattgccatcatgtacgtttttatctactgtcttaacgcccatgggaacggaggcgtcgtcgtcatgtattggacggcaacataggcagcaacacaaattgcgtttaggtggggtgcatgtggactcgataccaagcccctgcagctggggaacgtctggtggagagccgataatttgatatacgcacgccatattactgtcgttgaagtacgccttatcttctatgttttcaaatttaggttcccaagtggacgtgagaagtgtttgtatctcacatggaatggcccaaggcattccagcccaggtgcctggtactttaatggcaaacaaacgttttggtagaggtattgattctattgcagttctgcagatatctgcagccccgagtatccacaggctatacgatacgttatcggaggcctccgattctagcattacatagccggtcagtagatcctgccattcggtagcgcaaccggctacatcttcaaacagtctcacaataaatgcatctctcgttcctgccaatccggaaccgggcataccactcccgcctgccgatttaattctcacaattgggcgatgccggcggggcaaaacgaatgtggatttggcaaaccgacacaggtctgctgtacggactaatatgggcacacccacatcattcttcagatgctccatgcattgttctatgagaaagatccatagggtggaggcagcgtcacgagatcgcccaggcaatcgatcgcattcgtctagtaaagtgacgagagttatcatgcacacacccat

SEQ ID NO: 21 - DNA, 5381 bp, artificial sequence
  plasmid pCD046+NDV-F wt for vHVT110
gagctcagggtatgatactcagctgttattgtggccgaccaggaggactccaatgcttagcattcataagaacgctagagatgctatttaacgatgtgctgtcgtctaaagaatttgtgcatttagcctttaaatgtaaaaccaatgacgcattcactacgctcgtgcgtgcaatttctgggccagggtatgcatattccataacagaaatcgacacttgagaagaggatctgactgtttgggataaaggtcgtttgggtctgtcctagcgatataatttatatgacgatatacattaaacatctgtgtgcagtacttaggtatttaatcatgtcgatgaaatgttatgtgtaaatatcggacaatatagataacgggcacgctgctattgtaacgtgcgcccgcgcgctagtgctgactaatagtgtggatgatgtatacagtatattacaaacggaaatgatacgtaataaattatgtactcttattgatttataaaaacatacatgcagtgttgctatgtcacataattagcctcgcccgtctacgctccactgaagataatgggctcccgctgttcaaaaaaatcagcgtgcgtcgataagactttggtgcagtctcttcggggtcgcaatttagatttgccgcatggagggtatctggggatttttgccaatgctggagcgacgactgtacgattcgtcccatcgggatctagcagaccaatgatgttgacacacatcggccatgcatgtacggacggtctattgcgcgagtttgttattttcgaaggacaagatggaagtgtatatggaaccgacaataatgttagtttgcatttcttagggcggaatctacatgatatcttatccaagcggggtatgagccagagagatgtgatggtcataaagggtaaattttttagatctgaaataacgcagttgcccaaacaacgatcgcgattaaaagaaaaatcggatggttcaattaggacatgcatggattctgtgcgcataaaccataaccgcagcactgttgggcacttcggtaactcaaatgcgaagcgttgcacgtctgcgataactacgcctactatgcacattgttactcctgcatcttaaaaatatatcctgtagtaattttcacagcaatgtcataacatcatctcgctaaagaatgacctgggattggagaagtaatgaatatttgcaaccaatgcattgaataaactaacattaaacgaattcaatagtggatcccccaactccgcccgttttatgactagaaccaatagtttttaatgccaaatgcactgaaatcccctaatttgcaaagccaaacgccccctatgtgagtaatacggggactttttacccaatttcccacgcggaaagccccctaatacactcatatggcatatgaatcagcacggtcatgcactctaatggcggcccatagggactttccacatagggggcgttcaccatttcccagcataggggtggtgactcaatggcctttacccaagtacattgggtcaatgggaggtaagccaatgggtttttcccattactggcaagcacactgagtcaaatgggactttccactgggttttgcccaagtacattgggtcaatgggaggtgagccaatgggaaaaacccattgctgccaagtacactgactcaatagggactttccaatgggtttttccattgttggcaagcatataaggtcaatgtgggtgagtcaatagggactttccattgtattctgcccagtacataaggtcaatagggggtgaatcaacaggaaagtcccattggagccaagtacactgcgtcaatagggactttccattgggttttgcccagtacataaggtcaataggggatgagtcaatgggaaaaacccattggagccaagtacactgactcaatagggactttccattgggttttgcccagtacataaggtcaatagggggtgagtcaacaggaaagttccattggagccaagtacattgagtcaatagggactttccaatgggttttgcccagtacataaggtcaatgggaggtaagccaatgggtttttcccattactggcacgtatactgagtcattagggactttccaatgggttttgcccagtacataaggtcaataggggtgaatcaacaggaaagtcccattggagccaagtacactgagtcaatagggactttccattgggttttgcccagtacaaaaggtcaatagggggtgagtcaatgggtttttcccattattggcacgtacataaggtcaataggggtgagtcattgggtttttccagccaatttaattaaaacgccatgtactttcccaccattgacgtcaatgggctattgaaactaatgcaacgtgacctttaaacggtactttcccatagctgattaatgggaaagtaccgttctcgagccaatacacgtcaatgggaagtgaaagggcagccaaaacgtaacaccgccccggttttcccctggaaattccatattggcacgcattctattggctgagctgcgttctacgtgggtataagaggcgcgaccagcgtcggtaccgtcgcagtcttcggtctgaccaccgtagaacgcagagctcctcgctgcaggcggccgcatgggctccaaaccttctaccaggatcccagcacctctgatgctgatcacccggattatgctgatattgggctgtatccgtccgacaagctctcttgacggcaggcctcttgcagctgcaggaattgtagtaacaggagataaggcagtcaatgtatacacttcgtctcagacagggtcaatcatagtcaagttgctcccgaatatgcccagggataaggaggcgtgtgcaaaagccccattagaggcatataacagaacactgactactttgctcactcctcttggcgactccatccgcaagatccaagggtctgtgtccacatctggaggaggcaagcaaggccgcctgataggtgctgttattggcagtgtagctcttggggttgcaacagcggcacagataacagcagctgcggccctaatacaagccaaccagaatgccgccaacatcctccggcttaaggagagcattgctgcaaccaatgaagctgtgcatgaagtcaccgacggattatcacaactatcagtggcagttgggaagatgcagcagtttgtcaatgaccagtttaataatacggcgcgagaattggactgtataaaaatcacacaacaggttggtgtagaactcaacctatacctaactgaattgactacagtattcgggccacagatcacctcccctgcattaactcagctgaccatccaggcactttataatttagctggtggcaatatggattacttattaactaagttaggtatagggaacaatcaactcagctcgttaattggtagcggcctgatcactggttaccctatactgtatgactcacagactcaactcttgggcatacaagtgaatttaccctcagtcgggaacttaaataatatgcgtgccacctatttggagaccttatctgtaagtacaaccaaaggatatgcctcagcacttgtcccgaaagtagtgacacaagtcggttccgtgatagaagagcttgacacctcatactgtatagagtccgatctggatttatattgtactagaatagtgacattccccatgtccccaggtatttattcctgtttgagcggcaacacatcagcttgcatgtattcaaagactgaaggcgcactcactacgccgtatatggcccttaaaggctcagttattgccaattgtaaaataacaacatgtagatgtacagaccctcctggtatcatatcgcaaaattatggagaagctgtatccctgatagatagacattcgtgcaatgtcttatcattagacgggataactctaaggctcagtggggaatttgatgcaacttatcaaaagaacatctcaatactagattctcaagtcatcgtgacaggcaatcttgatatatcaactgaacttggaaacgtcaacaattcaatcagcaatgccttggataggttggcagaaagcaacagcaagctagaaaaagtcaatgtcagactaaccagcacatctgctctcattacctatattgttctaactgtcatttctctagttttcggtgcacttagtctggtgttagcgtgttacctgatgtacaaacagaaggcacaacaaaagaccttgctatggcttgggaataataccctcgatcagatgagagccactacaagagcatgagcggccgcggggatccagacatgataagatacattgatgagtttggacaaaccacaactagaatgcagtgaaaaaaatgctttatttgtgaaatttgtgatgctattgctttatttgtaaccattataagctgcaataaacaagttaacaacaacaattgcattgattttatgtttcaggttcagggggaggtgtgggaggttttttcggatcctctagagtcgacaattattttatttaataacatatagcccaaagacctctatgaacatttagtttcccgtatactcaacggcgcgtgtacacacgcatctctttgcatagcgatgaagtttgttcggcagcagaaaatgcagatatccaacaatctggagaaaacttatcatcacagtggcagtggaaacataccccctctatattcatggtataattatcgtctacagcgtccaggatagtggcgtgagaaaatggagatctgcagccctcctttccatggcatgccgctttattgttcattaaacgcacaatggtctcaacgccagatatgggcatagattctgaagaacccgttgacaatccgaagaagaaggcgtgcaggtctttggaagactcgcacgttggtcttataatgtatgatcgagatgtcaccctaatgccacatggtacaggcttatcgcggtcatggcgatcggacttgtaatttgcaacgatgggcaaaggatcgacgacatgccaaacattctgaacccgtagagatgttaacgatgacgaggatgaatatcccatgctcgctgccatagtatcaagtacaccgcgaataaggacgcgtccaacatcgttatatgcacacaatgggctacacgtgactaacacccccgaatattagtcatatgtgagtttcagtctggctcccatatagcctgtagactatttgtggtttaagtgtgaacgaggcgctgtgaacgagactcgggccgattgtaagaacaagcaaatgcactttccatttaacaagaagtgtagagagaatactcaacctctttggatgtatcctcgag

SEQ ID NO: 22 - DNA, 4337 bp, artificial sequence
  Partial plasmid pHM103+NDV-F wt sequence for vHVT111
gagctcagggtatgatactcagctgttattgtggccgaccaggaggactccaatgcttagcattcataagaacgctagagatgctatttaacgatgtgctgtcgtctaaagaatttgtgcatttagcctttaaatgtaaaaccaatgacgcattcactacgctcgtgcgtgcaatttctgggccagggtatgcatattccataacagaaatcgacacttgagaagaggatctgactgtttgggataaaggtcgtttgggtctgtcctagcgatataatttatatgacgatatacattaaacatctgtgtgcagtacttaggtatttaatcatgtcgatgaaatgttatgtgtaaatatcggacaatatagataacgggcacgctgctattgtaacgtgcgcccgcgcgctagtgctgactaatagtgtggatgatgtatacagtatattacaaacggaaatgatacgtaataaattatgtactcttattgatttataaaaacatacatgcagtgttgctatgtcacataattagcctcgcccgtctacgctccactgaagataatgggctcccgctgttcaaaaaaatcagcgtgcgtcgataagactttggtgcagtctcttcggggtcgcaatttagatttgccgcatggagggtatctggggatttttgccaatgctggagcgacgactgtacgattcgtcccatcgggatctagcagaccaatgatgttgacacacatcggccatgcatgtacggacggtctattgcgcgagtttgttattttcgaaggacaagatggaagtgtatatggaaccgacaataatgttagtttgcatttcttagggcggaatctacatgatatcttatccaagcggggtatgagccagagagatgtgatggtcataaagggtaaattttttagatctgaaataacgcagttgcccaaacaacgatcgcgattaaaagaaaaatcggatggttcaattaggacatgcatggattctgtgcgcataaaccataaccgcagcactgttgggcacttcggtaactcaaatgcgaagcgttgcacgtctgcgataactacgcctactatgcacattgttactcctgcatcttaaaaatatatcctgtagtaattttcacagcaatgtcataacatcatctcgctaaagaatgacctgggattggagaagtaatgaatatttgcaaccaatgcattgaataaactaacattaaacgaattcgagctcggtacagcttggctgtggaatgtgtgtcagttagggtgtggaaagtccccaggctccccagcaggcagaagtatgcaaagcatgcatctcaattagtcagcaaccaggtgtggaaagtccccaggctccccagcaggcagaagtatgcaaagcatgcatctcaattagtcagcaaccatagtcccgcccctaactccgcccatcccgcccctaactccgcccagttccgcccattctccgccccatggctgactaattttttttatttatgcagaggccgaggccgcctcggcctctgagctattccagaagtagtgaggaggcttttttggaggcctaggcttttgcaaaaagctgcggccgcatgggctccaaaccttctaccaggatcccagcacctctgatgctgatcacccggattatgctgatattgggctgtatccgtccgacaagctctcttgacggcaggcctcttgcagctgcaggaattgtagtaacaggagataaggcagtcaatgtatacacttcgtctcagacagggtcaatcatagtcaagttgctcccgaatatgcccagggataaggaggcgtgtgcaaaagccccattagaggcatataacagaacactgactactttgctcactcctcttggcgactccatccgcaagatccaagggtctgtgtccacatctggaggaggcaagcaaggccgcctgataggtgctgttattggcagtgtagctcttggggttgcaacagcggcacagataacagcagctgcggccctaatacaagccaaccagaatgccgccaacatcctccggcttaaggagagcattgctgcaaccaatgaagctgtgcatgaagtcaccgacggattatcacaactatcagtggcagttgggaagatgcagcagtttgtcaatgaccagtttaataatacggcgcgagaattggactgtataaaaatcacacaacaggttggtgtagaactcaacctatacctaactgaattgactacagtattcgggccacagatcacctcccctgcattaactcagctgaccatccaggcactttataatttagctggtggcaatatggattacttattaactaagttaggtatagggaacaatcaactcagctcgttaattggtagcggcctgatcactggttaccctatactgtatgactcacagactcaactcttgggcatacaagtgaatttaccctcagtcgggaacttaaataatatgcgtgccacctatttggagaccttatctgtaagtacaaccaaaggatatgcctcagcacttgtcccgaaagtagtgacacaagtcggttccgtgatagaagagcttgacacctcatactgtatagagtccgatctggatttatattgtactagaatagtgacattccccatgtccccaggtatttattcctgtttgagcggcaacacatcagcttgcatgtattcaaagactgaaggcgcactcactacgccgtatatggcccttaaaggctcagttattgccaattgtaaaataacaacatgtagatgtacagaccctcctggtatcatatcgcaaaattatggagaagctgtatccctgatagatagacattcgtgcaatgtcttatcattagacgggataactctaaggctcagtggggaatttgatgcaacttatcaaaagaacatctcaatactagattctcaagtcatcgtgacaggcaatcttgatatatcaactgaacttggaaacgtcaacaattcaatcagcaatgccttggataggttggcagaaagcaacagcaagctagaaaaagtcaatgtcagactaaccagcacatctgctctcattacctatattgttctaactgtcatttctctagttttcggtgcacttagtctggtgttagcgtgttacctgatgtacaaacagaaggcacaacaaaagaccttgctatggcttgggaataataccctcgatcagatgagagccactacaagagcatgagcggccgcggggatccagacatgataagatacattgatgagtttggacaaaccacaactagaatgcagtgaaaaaaatgctttatttgtgaaatttgtgatgctattgctttatttgtaaccattataagctgcaataaacaagttaacaacaacaattgcattgattttatgtttcaggttcagggggaggtgtgggaggttttttcggatcctctagagtcgacaattattttatttaataacatatagcccaaagacctctatgaacatttagtttcccgtatactcaacggcgcgtgtacacacgcatctctttgcatagcgatgaagtttgttcggcagcagaaaatgcagatatccaacaatctggagaaaacttatcatcacagtggcagtggaaacataccccctctatattcatggtataattatcgtctacagcgtccaggatagtggcgtgagaaaatggagatctgcagccctcctttccatggcatgccgctttattgttcattaaacgcacaatggtctcaacgccagatatgggcatagattctgaagaacccgttgacaatccgaagaagaaggcgtgcaggtctttggaagactcgcacgttggtcttataatgtatgatcgagatgtcaccctaatgccacatggtacaggcttatcgcggtcatggcgatcggacttgtaatttgcaacgatgggcaaaggatcgacgacatgccaaacattctgaacccgtagagatgttaacgatgacgaggatgaatatcccatgctcgctgccatagtatcaagtacaccgcgaataaggacgcgtccaacatcgttatatgcacacaatgggctacacgtgactaacacccccgaatattagtcatatgtgagtttcagtctggctcccatatagcctgtagactatttgtggtttaagtgtgaacgaggcgctgtgaacgagactcgggccgattgtaagaacaagcaaatgcactttccatttaacaagaagtgtagagagaatactcaacctctttggatgtatcctcgag

SEQ ID NO: 23 - DNA, 4344 bp, artificial sequence
  Partial plasmid pHM103+NDV-F CA02 for vHVT116
gagctcagggtatgatactcagctgttattgtggccgaccaggaggactccaatgcttagcattcataagaacgctagagatgctatttaacgatgtgctgtcgtctaaagaatttgtgcatttagcctttaaatgtaaaaccaatgacgcattcactacgctcgtgcgtgcaatttctgggccagggtatgcatattccataacagaaatcgacacttgagaagaggatctgactgtttgggataaaggtcgtttgggtctgtcctagcgatataatttatatgacgatatacattaaacatctgtgtgcagtacttaggtatttaatcatgtcgatgaaatgttatgtgtaaatatcggacaatatagataacgggcacgctgctattgtaacgtgcgcccgcgcgctagtgctgactaatagtgtggatgatgtatacagtatattacaaacggaaatgatacgtaataaattatgtactcttattgatttataaaaacatacatgcagtgttgctatgtcacataattagcctcgcccgtctacgctccactgaagataatgggctcccgctgttcaaaaaaatcagcgtgcgtcgataagactttggtgcagtctcttcggggtcgcaatttagatttgccgcatggagggtatctggggatttttgccaatgctggagcgacgactgtacgattcgtcccatcgggatctagcagaccaatgatgttgacacacatcggccatgcatgtacggacggtctattgcgcgagtttgttattttcgaaggacaagatggaagtgtatatggaaccgacaataatgttagtttgcatttcttagggcggaatctacatgatatcttatccaagcggggtatgagccagagagatgtgatggtcataaagggtaaattttttagatctgaaataacgcagttgcccaaacaacgatcgcgattaaaagaaaaatcggatggttcaattaggacatgcatggattctgtgcgcataaaccataaccgcagcactgttgggcacttcggtaactcaaatgcgaagcgttgcacgtctgcgataactacgcctactatgcacattgttactcctgcatcttaaaaatatatcctgtagtaattttcacagcaatgtcataacatcatctcgctaaagaatgacctgggattggagaagtaatgaatatttgcaaccaatgcattgaataaactaacattaaacgaattcgagctcggtacagcttggctgtggaatgtgtgtcagttagggtgtggaaagtccccaggctccccagcaggcagaagtatgcaaagcatgcatctcaattagtcagcaaccaggtgtggaaagtccccaggctccccagcaggcagaagtatgcaaagcatgcatctcaattagtcagcaaccatagtcccgcccctaactccgcccatcccgcccctaactccgcccagttccgcccattctccgccccatggctgactaattttttttatttatgcagaggccgaggccgcctcggcctctgagctattccagaagtagtgaggaggcttttttggaggcctaggcttttgcaaaaagctgcggccgccaccatgggcagcaagcccagcacctggatcagcgtgaccctgatgctgatcaccagaaccatgctgatcctgagctgcatctgccccacaagcagcctggacggcagacccctggccgctgccggcatcgtggtgaccggcgacaaggccgtgaacatctacaccagcagccagaccggcagcatcatcatcaagctgctgcccaacatgcccaaggacaaagaggcctgcgccaaggcccccctggaagcctacaacagaaccctgaccaccctgctgacccccctgggcgacagcatcagaagaatccagggcagcgccaccacaagcggcggaggaaagcagggcagactggtgggcgctatcatcgggagcgtggccctgggcgtggccacagctgcccagattaccgctgcagccgccctgattcaggccaatcagaacgccgccaacatcctgagactgaaagagagcattgccgccaccaacgacgccgtgcacgaagtgacaaacggactgtcccagctggctgtcgctgtcggcaagatgcagcagttcgtgaacaaccagttcaacaacaccgccagagagctggactgcatcaagatcgcccagcaggtgggcgtggagctgaacctgtacctgaccgagctgaccacagtgttcggcccccagatcacaagccccgctctgacccagctgacaatccaggccctgtacaacctggctggcggcaacatggactatctgctgactaagctgggagtgggcaacaaccagctgtccagcctgatcgggtccgggctgatcacaggcaaccccatcctgtacgacagccagacacagctgctgggcatccagatcaacctgccatccgtgggaagcctgaacaacatgagagccacctacctggaaaccctgagcgtgtccaccaccaagggcttcgccagcgccctggtgcccaaggtggtgacacaggtgggcagcgtgatcgaggaactggacaccagctactgcatcgagagcgacatcgacctgtactgcaccagagtggtgaccttcccaatgagccccggcatctacagctgcctgagcggcaacaccagcgcctgcatgtacagcaagaccgaaggagcactgacaacaccctacatggccctgaagggaagcgtgatcgccaactgcaagatgaccacctgcagatgcgccgaccccccaggcatcatcagccagaactacggcgaggccgtgagcctgatcgacaaacattcctgtagcgtgctgtccctggatggcatcacactgagactgagcggcgagttcgacgccacctaccagaagaacatcagcatcctggacagccaggtgatcgtgaccggcaacctggacatcagcaccgagctgggcaacgtgaacaacagcatcagcagcaccctggacaagctggccgagtccaacaacaagctgaacaaagtgaacgtgaacctgaccagcacaagcgccctgatcacctacatcgtgctggccatcgtgtccctggccttcggcgtgatcagcctggtgctggcctgctacctgatgtacaagcagagagcccagcagaaaaccctgctgtggctgggcaataacaccctggaccagatgagggccaccaccagaacctgatgagcggccgcggggatccagacatgataagatacattgatgagtttggacaaaccacaactagaatgcagtgaaaaaaatgctttatttgtgaaatttgtgatgctattgctttatttgtaaccattataagctgcaataaacaagttaacaacaacaattgcattgattttatgtttcaggttcagggggaggtgtgggaggttttttcggatcctctagagtcgacaattattttatttaataacatatagcccaaagacctctatgaacatttagtttcccgtatactcaacggcgcgtgtacacacgcatctctttgcatagcgatgaagtttgttcggcagcagaaaatgcagatatccaacaatctggagaaaacttatcatcacagtggcagtggaaacataccccctctatattcatggtataattatcgtctacagcgtccaggatagtggcgtgagaaaatggagatctgcagccctcctttccatggcatgccgctttattgttcattaaacgcacaatggtctcaacgccagatatgggcatagattctgaagaacccgttgacaatccgaagaagaaggcgtgcaggtctttggaagactcgcacgttggtcttataatgtatgatcgagatgtcaccctaatgccacatggtacaggcttatcgcggtcatggcgatcggacttgtaatttgcaacgatgggcaaaggatcgacgacatgccaaacattctgaacccgtagagatgttaacgatgacgaggatgaatatcccatgctcgctgccatagtatcaagtacaccgcgaataaggacgcgtccaacatcgttatatgcacacaatgggctacacgtgactaacacccccgaatattagtcatatgtgagtttcagtctggctcccatatagcctgtagactatttgtggtttaagtgtgaacgaggcgctgtgaacgagactcgggccgattgtaagaacaagcaaatgcactttccatttaacaagaagtgtagagagaatactcaacctctttggatgtatcctcgag

SEQ ID NO: 24 - DNA, 3988 bp, artificial sequence
  Partial plasmid HVTIG2 SV Fwt SbfI sequence for vHVT301
tgtttcgcaccatatccaagctggctgtccctaagagcttattcctgcaagacctcatacggaataattgcccgaccaatacttattacggacataggtaggccgataaatattatgttgactggaggatggaaaggaggttttgtaacagctacatcgctcgttcatcagcaagcgatactttggatatccgagcttcaaaagccgcataaaccccgctttatttctgaatacgccccaacagtaacacatgcgtggttcctggcacttggaacgccgtgttttataggcaagaacatactacccaaagaggtcttgggatttctggcgcgtcgttgcaatgaagaaatgaattctttgttccttgaaatgccgacaactctaaaaacggtattcgagcaccattactttacgcgtggatctgaagtaaatccagcgttgttgatggagcctaacagatttttgcaactgatggattcgcggaaaatcctatgtttatacgaatccgctatgtgcgacaaccccggagctcagggtatgatactcagctgttattgtggccgaccaggaggactccaatgcttagcattcataagaacgctagagatgctatttaacgatgtgctgtcgtctaaagaatttgtgcatttagcctttaaatgtaaaaccaatgacgcattcactacgctcgtgcgtgcaatttctgggccagggtatgcatattccataacagaaatcgacacttgagaagaggatctgactgtttgggataaaggtcgtttgggtctgtcctagcgatataatttatatgacgatatacattaaacatctgtgtgcagtacttaggtatttaatcatgtcgatgaaatgttatgtgtaaatatcggacaatatagataacgggcacgctgctattgtaacgtgcgcccgcgcgctagtgctgactaatagtgtggatgatgtatacagtatattacaaacggaaatgatacgtaataaacctgcaggtcgacccaattcgagctcggtacagcttggctgtggaatgtgtgtcagttagggtgtggaaagtccccaggctccccagcaggcagaagtatgcaaagcatgcatctcaattagtcagcaaccaggtgtggaaagtccccaggctccccagcaggcagaagtatgcaaagcatgcatctcaattagtcagcaaccatagtcccgcccctaactccgcccatcccgcccctaactccgcccagttccgcccattctccgccccatggctgactaattttttttatttatgcagaggccgaggccgcctcggcctctgagctattccagaagtagtgaggaggcttttttggaggcctaggcttttgcaaaaagctgcggccgcatgggctccaaaccttctaccaggatcccagcacctctgatgctgatcacccggattatgctgatattgggctgtatccgtccgacaagctctcttgacggcaggcctcttgcagctgcaggaattgtagtaacaggagataaggcagtcaatgtatacacttcgtctcagacagggtcaatcatagtcaagttgctcccgaatatgcccagggataaggaggcgtgtgcaaaagccccattagaggcatataacagaacactgactactttgctcactcctcttggcgactccatccgcaagatccaagggtctgtgtccacatctggaggaggcaagcaaggccgcctgataggtgctgttattggcagtgtagctcttggggttgcaacagcggcacagataacagcagctgcggccctaatacaagccaaccagaatgccgccaacatcctccggcttaaggagagcattgctgcaaccaatgaagctgtgcatgaagtcaccgacggattatcacaactatcagtggcagttgggaagatgcagcagtttgtcaatgaccagtttaataatacggcgcgagaattggactgtataaaaatcacacaacaggttggtgtagaactcaacctatacctaactgaattgactacagtattcgggccacagatcacctcccctgcattaactcagctgaccatccaggcactttataatttagctggtggcaatatggattacttattaactaagttaggtatagggaacaatcaactcagctcgttaattggtagcggcctgatcactggttaccctatactgtatgactcacagactcaactcttgggcatacaagtgaatttaccctcagtcgggaacttaaataatatgcgtgccacctatttggagaccttatctgtaagtacaaccaaaggatatgcctcagcacttgtcccgaaagtagtgacacaagtcggttccgtgatagaagagcttgacacctcatactgtatagagtccgatctggatttatattgtactagaatagtgacattccccatgtccccaggtatttattcctgtttgagcggcaacacatcagcttgcatgtattcaaagactgaaggcgcactcactacgccgtatatggcccttaaaggctcagttattgccaattgtaaaataacaacatgtagatgtacagaccctcctggtatcatatcgcaaaattatggagaagctgtatccctgatagatagacattcgtgcaatgtcttatcattagacgggataactctaaggctcagtggggaatttgatgcaacttatcaaaagaacatctcaatactagattctcaagtcatcgtgacaggcaatcttgatatatcaactgaacttggaaacgtcaacaattcaatcagcaatgccttggataggttggcagaaagcaacagcaagctagaaaaagtcaatgtcagactaaccagcacatctgctctcattacctatattgttctaactgtcatttctctagttttcggtgcacttagtctggtgttagcgtgttacctgatgtacaaacagaaggcacaacaaaagaccttgctatggcttgggaataataccctcgatcagatgagagccactacaagagcatgagcggccgcggggatccagacatgataagatacattgatgagtttggacaaaccacaactagaatgcagtgaaaaaaatgctttatttgtgaaatttgtgatgctattgctttatttgtaaccattataagctgcaataaacaagttaacaacaacaattgcattgattttatgtttcaggttcagggggaggtgtgggaggttttttcggatcctctagaggggattaatcctgcaggttatgtactcttattgatttataaaaacatacatgcagtgttgctatgtcacataattagcctcgcccgtctacgctccactgaagataatgggctcccgctgttcaaaaaaatcagcgtgcgtcgataagactttggtgcagtctcttcggggtcgcaatttagatttgccgcatggagggtatctggggatttttgccaatgctggagcgacgactgtacgattcgtcccatcgggatctagcagaccaatgatgttgacacacatcggccatgcatgtacggacggtctattgcgcgagtttgttattttcgaaggacaagatggaagtgtatatggaaccgacaataatgttagtttgcatttcttagggcggaatctacatgatatcttatccaagcggggtatgagccagagagatgtgatggtcataaagggtaaattttttagatctgaaataacgcagttgcccaaacaacgatcgcgattaaaagaaaaatcggatggttcaattaggacatgcatggattctgtgcgcataaaccataaccgcagcactgttgggcacttcggtaactcaaatgcgaagcgttgcacgtctgcgataactacgcctactatgcacattgttactcctgcatcttaaaaatatatcctgtagtaattttcacagcaatgtcataacatcatctcgcta

SEQ ID NO: 25 - DNA, 3707 bp, artificial sequence
  Partial plasmid pHVTUS10 cds F opt plasmid for vHVT302
tcccttacggcggatcgaaacgacattaggcatactcgggtaccattttgcattccgatcagcacggatgaaattaggcaggaatgcggtttatattatgcggcattggacaaacgatatggcattgattggcagtttatgaatgtcttcatgttgggcgtaaacggattcctattggttcagaagacaacgacgatatatttagagagaaaaagctacccagcataggataaacacacattgagcattgagagacataggtatcggtatggatgggaaaactacacacgtgaacaccaaacgacttatatactcgagcggtgatactactgagcaagaatgcactgcatctgagccactgaatgaagactgtgatgaaaatgtgaccatcgatggaattggagaagaatatgcgcagttcttcatgtccccgcaatgggtcccaaatctacatcgcttgagcgaggataccaaaaaggtataccgatgtatggtttccaacagactcaattattttccctattatgaggcgttcaggcggtctttgtttgatatgtatatgctaggtcggttggggcgtcgacttaagcgatctgactgggagactattatgcatctgtcaccaacgcaaagtcggcgtctacatagaactttaagatttgtggagcgtagaattatcccatctaacagttatatacgcacatcgggccacgttccgccttcgagggcacttccgacagatacgaatttaaagatggatgaataattaaattggaaagagtaactacattaatcgagcgtcatgacggcgtcccgtgaaaatgggaattttctactcgaaacaccgtgacatttgacagacctggaattgttattctgatatatagtgggtgtgtctggccggcaacatacataatgtgcatgcgaaaccactttttcagtgtacgctgacattgtgcaacacggaggggtagcatctacatacaatatatgttgattacctgcagggcggccgccaccatgggcagcaagcccagcacaagaatcccagcccccctgatgctgatcacccgcatcatgctgatcctgggctgcatcagacccacaagctccctggatggacgccccctggccgctgccggcatcgtggtgaccggcgacaaggccgtgaacgtgtacaccagcagccagaccggcagcatcatcgtgaagctgctgcccaacatgcccagagacaaagaggcctgcgccaaggcccccctggaagcctacaacagaaccctgaccaccctgctgacccccctgggcgacagcatcagaaagatccagggctccgtgagcacaagcggcggaggaaagcagggcagactgatcggcgccgtgatcggcagcgtggccctgggagtggctacagctgcccagattaccgctgcagccgccctgatccaggccaaccagaacgccgccaacatcctgagactgaaagagagcattgccgccaccaacgaggccgtgcacgaagtgaccgacggcctgagccagctgtccgtggccgtgggcaagatgcagcagttcgtgaacgaccagttcaacaacaccgccagagagctggactgcatcaagatcacccagcaggtgggcgtggagctgaacctgtacctgaccgagctgaccacagtgttcggcccccagatcacaagcccagccctgacacagctgaccatccaggccctgtacaacctggctggcggcaacatggactatctgctgacaaagctgggaatcggcaacaaccagctgtccagcctgatcggaagcggcctgatcaccggctaccccatcctgtacgacagccagacacagctgctgggcatccaggtgaacctgcccagcgtgggcaacctgaacaacatgcgcgccacctacctggaaaccctgagcgtgtccaccaccaagggctacgccagcgccctggtgcccaaggtggtgacacaggtgggcagcgtgatcgaggaactggacaccagctactgcatcgagagcgacctggacctgtactgcaccagaatcgtgaccttcccaatgagccccggcatctacagctgcctgagcggcaacaccagcgcctgcatgtacagcaagaccgaaggcgcactgacaacaccctacatggccctgaagggaagcgtgatcgccaactgcaagatcaccacctgcagatgcaccgaccccccaggcatcatcagccagaactacggcgaggccgtgagcctgatcgatcgccattcctgtaacgtgctgtccctggacggcatcacactgagactgagcggcgagttcgatgccacctaccagaagaacatcagcatcctggacagccaggtgatcgtgaccggcaacctggacatcagcaccgagctgggcaacgtgaataacagcatcagcaacgccctggacagactggccgagagcaacagcaagctggaaaaagtgaacgtgcgcctgacatccacttccgctctgatcacctacatcgtgctgaccgtgatcagcctggtgttcggcgccctgagcctggtgctggcctgctacctgatgtacaagcagaaggcccagcagaaaaccctgctgtggctgggcaacaacaccctggaccagatgagagccaccaccagagcctgatgagcggccgccccgggcctgcaggcataggcacgctctgatgttacagaccacaataccgcatacatttattgtaaggttgttaataaaggtttattctatgtaagactacaatactttcgacattgcttgtatacatattaaatactttctcaagttcctattacataaaatgggatctatcattacattcgttaagagtctggataattttactgtttgccagcttcgatcttggaacgtactgtggatagtgccttacttggaatcgtgaaaatttgaaacgtccattatttggatatcttccggttgtcccatatcccgccctggtaccgctcggataccttgcccgtatggattcgtattgacagtcgcgcaatcggggaccaacaacgcgtgggtccacactcattcggaaattttccgatgattctgaatatttattgccgctcgttacgagtcgttggacatatctgtaatacatttcttcttctgaaggatcgctgcacatttgatctatacattggccaggatgttcaagtctcagatgttgcattctggcacagcacaactttatggcatttccgatgtaatcgtccggcagccctgggggagttctatattcgcatattgggatggtaaggacaatagcagatctcgcaacctccagggaggctataataacgtttttaaaggatggatttctcataaaaatctgtcgcaaattacactgagaatatcctttactagcgccgattgagagcatcgtcgtccaattttctaaatggaaagaaaacaaggcgggcaagagtgttccaaacattttcattttcggcgaatctctcaaatcccatggcgtgcaattgattgcaaaattggcacttccgttcacgtttgtatctccaaactctaagacacttttaattgaaaaactacgttctagtgtggaaagaaacctataggcagaccatagaactatttgacaccacatatctttttgtatgtcaaactgaccatgatcgtat

SEQ ID NO: 26 - DNA, 3707 bp, artificial sequence
  Partial plasmid pHVT US20 cds F CA02 opt sequence for vHVT303
tcccttacggcggatcgaaacgacattaggcatactcgggtaccattttgcattccgatcagcacggatgaaattaggcaggaatgcggtttatattatgcggcattggacaaacgatatggcattgattggcagtttatgaatgtcttcatgttgggcgtaaacggattcctattggttcagaagacaacgacgatatatttagagagaaaaagctacccagcataggataaacacacattgagcattgagagacataggtatcggtatggatgggaaaactacacacgtgaacaccaaacgacttatatactcgagcggtgatactactgagcaagaatgcactgcatctgagccactgaatgaagactgtgatgaaaatgtgaccatcgatggaattggagaagaatatgcgcagttcttcatgtccccgcaatgggtcccaaatctacatcgcttgagcgaggataccaaaaaggtataccgatgtatggtttccaacagactcaattattttccctattatgaggcgttcaggcggtctttgtttgatatgtatatgctaggtcggttggggcgtcgacttaagcgatctgactgggagactattatgcatctgtcaccaacgcaaagtcggcgtctacatagaactttaagatttgtggagcgtagaattatcccatctaacagttatatacgcacatcgggccacgttccgccttcgagggcacttccgacagatacgaatttaaagatggatgaataattaaattggaaagagtaactacattaatcgagcgtcatgacggcgtcccgtgaaaatgggaattttctactcgaaacaccgtgacatttgacagacctggaattgttattctgatatatagtgggtgtgtctggccggcaacatacataatgtgcatgcgaaaccactttttcagtgtacgctgacattgtgcaacacggaggggtagcatctacatacaatatatgttgattacctgcagggcggccgccaccatgggcagcaagcccagcacctggatcagcgtgaccctgatgctgatcaccagaaccatgctgatcctgagctgcatctgccccacaagcagcctggacggcagacccctggccgctgccggcatcgtggtgaccggcgacaaggccgtgaacatctacaccagcagccagaccggcagcatcatcatcaagctgctgcccaacatgcccaaggacaaagaggcctgcgccaaggcccccctggaagcctacaacagaaccctgaccaccctgctgacccccctgggcgacagcatcagaagaatccagggcagcgccaccacaagcggcggaggaaagcagggcagactggtgggcgctatcatcgggagcgtggccctgggcgtggccacagctgcccagattaccgctgcagccgccctgattcaggccaatcagaacgccgccaacatcctgagactgaaagagagcattgccgccaccaacgacgccgtgcacgaagtgacaaacggactgtcccagctggctgtcgctgtcggcaagatgcagcagttcgtgaacaaccagttcaacaacaccgccagagagctggactgcatcaagatcgcccagcaggtgggcgtggagctgaacctgtacctgaccgagctgaccacagtgttcggcccccagatcacaagccccgctctgacccagctgacaatccaggccctgtacaacctggctggcggcaacatggactatctgctgactaagctgggagtgggcaacaaccagctgtccagcctgatcgggtccgggctgatcacaggcaaccccatcctgtacgacagccagacacagctgctgggcatccagatcaacctgccatccgtgggaagcctgaacaacatgagagccacctacctggaaaccctgagcgtgtccaccaccaagggcttcgccagcgccctggtgcccaaggtggtgacacaggtgggcagcgtgatcgaggaactggacaccagctactgcatcgagagcgacatcgacctgtactgcaccagagtggtgaccttcccaatgagccccggcatctacagctgcctgagcggcaacaccagcgcctgcatgtacagcaagaccgaaggagcactgacaacaccctacatggccctgaagggaagcgtgatcgccaactgcaagatgaccacctgcagatgcgccgaccccccaggcatcatcagccagaactacggcgaggccgtgagcctgatcgacaaacattcctgtagcgtgctgtccctggatggcatcacactgagactgagcggcgagttcgacgccacctaccagaagaacatcagcatcctggacagccaggtgatcgtgaccggcaacctggacatcagcaccgagctgggcaacgtgaacaacagcatcagcagcaccctggacaagctggccgagtccaacaacaagctgaacaaagtgaacgtgaacctgaccagcacaagcgccctgatcacctacatcgtgctggccatcgtgtccctggccttcggcgtgatcagcctggtgctggcctgctacctgatgtacaagcagagagcccagcagaaaaccctgctgtggctgggcaataacaccctggaccagatgagggccaccaccagaacctgatgagcggccgccccgggcctgcaggcataggcacgctctgatgttacagaccacaataccgcatacatttattgtaaggttgttaataaaggtttattctatgtaagactacaatactttcgacattgcttgtatacatattaaatactttctcaagttcctattacataaaatgggatctatcattacattcgttaagagtctggataattttactgtttgccagcttcgatcttggaacgtactgtggatagtgccttacttggaatcgtgaaaatttgaaacgtccattatttggatatcttccggttgtcccatatcccgccctggtaccgctcggataccttgcccgtatggattcgtattgacagtcgcgcaatcggggaccaacaacgcgtgggtccacactcattcggaaattttccgatgattctgaatatttattgccgctcgttacgagtcgttggacatatctgtaatacatttcttcttctgaaggatcgctgcacatttgatctatacattggccaggatgttcaagtctcagatgttgcattctggcacagcacaactttatggcatttccgatgtaatcgtccggcagccctgggggagttctatattcgcatattgggatggtaaggacaatagcagatctcgcaacctccagggaggctataataacgtttttaaaggatggatttctcataaaaatctgtcgcaaattacactgagaatatcctttactagcgccgattgagagcatcgtcgtccaattttctaaatggaaagaaaacaaggcgggcaagagtgttccaaacattttcattttcggcgaatctctcaaatcccatggcgtgcaattgattgcaaaattggcacttccgttcacgtttgtatctccaaactctaagacacttttaattgaaaaactacgttctagtgtggaaagaaacctataggcagaccatagaactatttgacaccacatatctttttgtatgtcaaactgaccatgatcgtat

SEQ ID NO: 27 - DNA, 3946 bp, artificial sequence
  Partial plasmid HVT IG2 SVFopt syn tail sequence for vHVT304
tgtttcgcaccatatccaagctggctgtccctaagagcttattcctgcaagacctcatacggaataattgcccgaccaatacttattacggacataggtaggccgataaatattatgttgactggaggatggaaaggaggttttgtaacagctacatcgctcgttcatcagcaagcgatactttggatatccgagcttcaaaagccgcataaaccccgctttatttctgaatacgccccaacagtaacacatgcgtggttcctggcacttggaacgccgtgttttataggcaagaacatactacccaaagaggtcttgggatttctggcgcgtcgttgcaatgaagaaatgaattctttgttccttgaaatgccgacaactctaaaaacggtattcgagcaccattactttacgcgtggatctgaagtaaatccagcgttgttgatggagcctaacagatttttgcaactgatggattcgcggaaaatcctatgtttatacgaatccgctatgtgcgacaaccccggagctcagggtatgatactcagctgttattgtggccgaccaggaggactccaatgcttagcattcataagaacgctagagatgctatttaacgatgtgctgtcgtctaaagaatttgtgcatttagcctttaaatgtaaaaccaatgacgcattcactacgctcgtgcgtgcaatttctgggccagggtatgcatattccataacagaaatcgacacttgagaagaggatctgactgtttgggataaaggtcgtttgggtctgtcctagcgatataatttatatgacgatatacattaaacatctgtgtgcagtacttaggtatttaatcatgtcgatgaaatgttatgtgtaaatatcggacaatatagataacgggcacgctgctattgtaacgtgcgcccgcgcgctagtgctgactaatagtgtggatgatgtatacagtatattacaaacggaaatgatacgtaataaacctgcaggtcgacccaattcgagctcggtacagcttggctgtggaatgtgtgtcagttagggtgtggaaagtccccaggctccccagcaggcagaagtatgcaaagcatgcatctcaattagtcagcaaccaggtgtggaaagtccccaggctccccagcaggcagaagtatgcaaagcatgcatctcaattagtcagcaaccatagtcccgcccctaactccgcccatcccgcccctaactccgcccagttccgcccattctccgccccatggctgactaattttttttatttatgcagaggccgaggccgcctcggcctctgagctattccagaagtagtgaggaggcttttttggaggcctaggcttttgcaaaaagctcccggggcggccgccaccatgggcagcaagcccagcacaagaatcccagcccccctgatgctgatcacccgcatcatgctgatcctgggctgcatcagacccacaagctccctggatggacgccccctggccgctgccggcatcgtggtgaccggcgacaaggccgtgaacgtgtacaccagcagccagaccggcagcatcatcgtgaagctgctgcccaacatgcccagagacaaagaggcctgcgccaaggcccccctggaagcctacaacagaaccctgaccaccctgctgacccccctgggcgacagcatcagaaagatccagggctccgtgagcacaagcggcggaggaaagcagggcagactgatcggcgccgtgatcggcagcgtggccctgggagtggctacagctgcccagattaccgctgcagccgccctgatccaggccaaccagaacgccgccaacatcctgagactgaaagagagcattgccgccaccaacgaggccgtgcacgaagtgaccgacggcctgagccagctgtccgtggccgtgggcaagatgcagcagttcgtgaacgaccagttcaacaacaccgccagagagctggactgcatcaagatcacccagcaggtgggcgtggagctgaacctgtacctgaccgagctgaccacagtgttcggcccccagatcacaagcccagccctgacacagctgaccatccaggccctgtacaacctggctggcggcaacatggactatctgctgacaaagctgggaatcggcaacaaccagctgtccagcctgatcggaagcggcctgatcaccggctaccccatcctgtacgacagccagacacagctgctgggcatccaggtgaacctgcccagcgtgggcaacctgaacaacatgcgcgccacctacctggaaaccctgagcgtgtccaccaccaagggctacgccagcgccctggtgcccaaggtggtgacacaggtgggcagcgtgatcgaggaactggacaccagctactgcatcgagagcgacctggacctgtactgcaccagaatcgtgaccttcccaatgagccccggcatctacagctgcctgagcggcaacaccagcgcctgcatgtacagcaagaccgaaggcgcactgacaacaccctacatggccctgaagggaagcgtgatcgccaactgcaagatcaccacctgcagatgcaccgaccccccaggcatcatcagccagaactacggcgaggccgtgagcctgatcgatcgccattcctgtaacgtgctgtccctggacggcatcacactgagactgagcggcgagttcgatgccacctaccagaagaacatcagcatcctggacagccaggtgatcgtgaccggcaacctggacatcagcaccgagctgggcaacgtgaataacagcatcagcaacgccctggacagactggccgagagcaacagcaagctggaaaaagtgaacgtgcgcctgacatccacttccgctctgatcacctacatcgtgctgaccgtgatcagcctggtgttcggcgccctgagcctggtgctggcctgctacctgatgtacaagcagaaggcccagcagaaaaccctgctgtggctgggcaacaacaccctggaccagatgagagccaccaccagagcctgatgagcggccgcgatatcaataaaatatctttattttcattacatctgtgtgttggttttttgtgtgaatcgatagtactaacatacgctctccatcaaaacaaaacgaaacaaaacaaactagcaaaataggctgtccccagtgcaagtgcaggtgccagaacatttctcttctagacctgcaggttatgtactcttattgatttataaaaacatacatgcagtgttgctatgtcacataattagcctcgcccgtctacgctccactgaagataatgggctcccgctgttcaaaaaaatcagcgtgcgtcgataagactttggtgcagtctcttcggggtcgcaatttagatttgccgcatggagggtatctggggatttttgccaatgctggagcgacgactgtacgattcgtcccatcgggatctagcagaccaatgatgttgacacacatcggccatgcatgtacggacggtctattgcgcgagtttgttattttcgaaggacaagatggaagtgtatatggaaccgacaataatgttagtttgcatttcttagggcggaatctacatgatatcttatccaagcggggtatgagccagagagatgtgatggtcataaagggtaaattttttagatctgaaataacgcagttgcccaaacaacgatcgcgattaaaagaaaaatcggatggttcaattaggacatgcatggattctgtgcgcataaaccataaccgcagcactgttgggcacttcggtaactcaaatgcgaagcgttgcacgtctgcgataactacgcctactatgcacattgttactcctgcatcttaaaaatatatcctgtagtaattttcacagcaatgtcataacatcatctcgctaa

SEQ ID NO: 28 - DNA, 4654 bp, artificial sequence
  Partial plasmid pHVT US2 SV-FCA02 opt-synPA for vHVT307
tatctccacatcgtattcaggcccacggaagtcttcgttatcgaagctattgttactagtatctggcgacatcgacggttctgcaaccgtcgtaccgctttcgatattttcacagacaatacccatattcgaggcacttactttcgaagactcaacatctacttccatcgccgccacgtatgtaatttcgggacgttggatgatataaaatatatagtacgcgtccgggtatacacctgtgcgaaagtagtacgagaccggcagtcaaaaagacgtttccgatcttccacagctccagttattcggaaggcgtgggcatgggtgtgtgcatgataactctcgtcactttactagacgaatgcgatcgattgcctgggcgatctcgtgacgctgcctccaccctatggatctttctcatagaacaatgcatggagcatctgaagaatgatgtgggtgtgcccatattagtccgtacagcagacctgtgtcggtttgccaaatccacattcgttttgccccgccggcatcgcccaattgtgagaattaaatcggcaggcgggagtggtatgcccggttccggattggcaggaacgagagatgcatttattgtgagactgtttgaagatgtagccggttgcgctaccgaatggcaggatctactgaccggctatgtaatgctagaatcggaggcctccgataacgtatcgtatagcctgtggatactcggggctgcagatatctgcagaactgcaatagaatcaatacctctaccaaaacgtttgtttgccattaaagtaccaggcacctgggctggaatgccttgggccattccatgtgagatacaaacacttctcacgtccacttgggaacctaaatttgaaaacatagaagataaggcgtacttcaacgacagtaatatggcgtgcgtatatcaaattatcggctctccaccagacgttccccagctgcaggggcttggtatcgagtccacatgcaccccacctaaacgcaatttgtgttgctgcctatgttgccgtccaatacatgacgacgacgcctccgttcccatgggcgttaagacagtagataaaaacgtacatgatggcaatatgcttgtagaggctcccaagtgtatcacagataggggaaaattcaatagtagataaacccaactagtgtgaggaaattgcatctacttgcccccgggcctgcaggtcgacccaattcgagctcggtacagcttggctgtggaatgtgtgtcagttagggtgtggaaagtccccaggctccccagcaggcagaagtatgcaaagcatgcatctcaattagtcagcaaccaggtgtggaaagtccccaggctccccagcaggcagaagtatgcaaagcatgcatctcaattagtcagcaaccatagtcccgcccctaactccgcccatcccgcccctaactccgcccagttccgcccattctccgccccatggctgactaattttttttatttatgcagaggccgaggccgcctcggcctctgagctattccagaagtagtgaggaggcttttttggaggcctaggcttttgcaaaaagctcccggggcggccgccaccatgggcagcaagcccagcacctggatcagcgtgaccctgatgctgatcaccagaaccatgctgatcctgagctgcatctgccccacaagcagcctggacggcagacccctggccgctgccggcatcgtggtgaccggcgacaaggccgtgaacatctacaccagcagccagaccggcagcatcatcatcaagctgctgcccaacatgcccaaggacaaagaggcctgcgccaaggcccccctggaagcctacaacagaaccctgaccaccctgctgacccccctgggcgacagcatcagaagaatccagggcagcgccaccacaagcggcggaggaaagcagggcagactggtgggcgctatcatcgggagcgtggccctgggcgtggccacagctgcccagattaccgctgcagccgccctgattcaggccaatcagaacgccgccaacatcctgagactgaaagagagcattgccgccaccaacgacgccgtgcacgaagtgacaaacggactgtcccagctggctgtcgctgtcggcaagatgcagcagttcgtgaacaaccagttcaacaacaccgccagagagctggactgcatcaagatcgcccagcaggtgggcgtggagctgaacctgtacctgaccgagctgaccacagtgttcggcccccagatcacaagccccgctctgacccagctgacaatccaggccctgtacaacctggctggcggcaacatggactatctgctgactaagctgggagtgggcaacaaccagctgtccagcctgatcgggtccgggctgatcacaggcaaccccatcctgtacgacagccagacacagctgctgggcatccagatcaacctgccatccgtgggaagcctgaacaacatgagagccacctacctggaaaccctgagcgtgtccaccaccaagggcttcgccagcgccctggtgcccaaggtggtgacacaggtgggcagcgtgatcgaggaactggacaccagctactgcatcgagagcgacatcgacctgtactgcaccagagtggtgaccttcccaatgagccccggcatctacagctgcctgagcggcaacaccagcgcctgcatgtacagcaagaccgaaggagcactgacaacaccctacatggccctgaagggaagcgtgatcgccaactgcaagatgaccacctgcagatgcgccgaccccccaggcatcatcagccagaactacggcgaggccgtgagcctgatcgacaaacattcctgtagcgtgctgtccctggatggcatcacactgagactgagcggcgagttcgacgccacctaccagaagaacatcagcatcctggacagccaggtgatcgtgaccggcaacctggacatcagcaccgagctgggcaacgtgaacaacagcatcagcagcaccctggacaagctggccgagtccaacaacaagctgaacaaagtgaacgtgaacctgaccagcacaagcgccctgatcacctacatcgtgctggccatcgtgtccctggccttcggcgtgatcagcctggtgctggcctgctacctgatgtacaagcagagagcccagcagaaaaccctgctgtggctgggcaataacaccctggaccagatgagggccaccaccagaacctgatgagcggccgcgatatcaataaaatatctttattttcattacatctgtgtgttggttttttgtgtgaatcgatagtactaacatacgctctccatcaaaacaaaacgaaacaaaacaaactagcaaaataggctgtccccagtgcaagtgcaggtgccagaacatttctcttctagacctgcaggcatatgttgtcccattatgttgtacataatcgtgatgtagtgctacgcaaatgtcaattgatagcccatacatggtgctaatatgcgttacttttagtatgtgagtgaataaaaaaatattacccctatgatacctgcgtctttatgctacaagttccttcaccatgaccagagccggtgcgatcatattcgacaacttggatattcccagaggtagatttggccagccgcggggaaaaataaatgacttcaactactggaccttgctaaccgatgagctgacgtgtggaattattcaatgtatggagtcgcgcgagcgaattgccctagtgcattcagcaacatacgatcatggtcagtttgacatacaaaaagatatgtggtgtcaaatagttctatggtctgcctataggtttctttccacactagaacgtagtttttcaattaaaagtgtcttagagtttggagatacaaacgtgaacggaagtgccaattttgcaatcaattgcacgccatgggatttgagagattcgccgaaaatgaaaatgtttggaacactcttgcccgccttgttttctttccatttagaaaattggacgacgatgctctcaatcggcgctagtaaaggatattctcagtgtaatttgcgacagatttttatgagaaatccatcctttaaaaacgttattatagcctccctggaggttgcgagatctgctattgtccttaccatcccaatatgcgaatatagaactcccccagggctgccggacgattacatcggaaatgccataaagttgtgctgtgccagaatgcaacatctgagacttgaacatcctggccaatgtatagatcaaatgtgcagcgatccttcagaagaagaaatgtattacagatatgtccaacgactcgtaacgagcggcaataaatattcagaatcatcggaaaatttccgaatgagtgtggacccacgcgttgttggtccccgattgcgcgactgtcaatacgaatccatacgggcaaggtatccgagcggtaccagggcgggatatgggacaaccggaagatatccaaataatggacgtttcaaattttcacgattccaagtaaggcactatccacagtacgttccaagatcgaagctggcaaacagtaaaattatccagactcttaacgaatgtaatgatagatcccatttta

SEQ ID NO: 29 - DNA, 5381 bp, artificial sequence
  partial plasmid pCD046+NDV-F VII YZCQ sequence for HVT112
gagctcagggtatgatactcagctgttattgtggccgaccaggaggactccaatgcttagcattcataagaacgctagagatgctatttaacgatgtgctgtcgtctaaagaatttgtgcatttagcctttaaatgtaaaaccaatgacgcattcactacgctcgtgcgtgcaatttctgggccagggtatgcatattccataacagaaatcgacacttgagaagaggatctgactgtttgggataaaggtcgtttgggtctgtcctagcgatataatttatatgacgatatacattaaacatctgtgtgcagtacttaggtatttaatcatgtcgatgaaatgttatgtgtaaatatcggacaatatagataacgggcacgctgctattgtaacgtgcgcccgcgcgctagtgctgactaatagtgtggatgatgtatacagtatattacaaacggaaatgatacgtaataaattatgtactcttattgatttataaaaacatacatgcagtgttgctatgtcacataattagcctcgcccgtctacgctccactgaagataatgggctcccgctgttcaaaaaaatcagcgtgcgtcgataagactttggtgcagtctcttcggggtcgcaatttagatttgccgcatggagggtatctggggatttttgccaatgctggagcgacgactgtacgattcgtcccatcgggatctagcagaccaatgatgttgacacacatcggccatgcatgtacggacggtctattgcgcgagtttgttattttcgaaggacaagatggaagtgtatatggaaccgacaataatgttagtttgcatttcttagggcggaatctacatgatatcttatccaagcggggtatgagccagagagatgtgatggtcataaagggtaaattttttagatctgaaataacgcagttgcccaaacaacgatcgcgattaaaagaaaaatcggatggttcaattaggacatgcatggattctgtgcgcataaaccataaccgcagcactgttgggcacttcggtaactcaaatgcgaagcgttgcacgtctgcgataactacgcctactatgcacattgttactcctgcatcttaaaaatatatcctgtagtaattttcacagcaatgtcataacatcatctcgctaaagaatgacctgggattggagaagtaatgaatatttgcaaccaatgcattgaataaactaacattaaacgaattcaatagtggatcccccaactccgcccgttttatgactagaaccaatagtttttaatgccaaatgcactgaaatcccctaatttgcaaagccaaacgccccctatgtgagtaatacggggactttttacccaatttcccacgcggaaagccccctaatacactcatatggcatatgaatcagcacggtcatgcactctaatggcggcccatagggactttccacatagggggcgttcaccatttcccagcataggggtggtgactcaatggcctttacccaagtacattgggtcaatgggaggtaagccaatgggtttttcccattactggcaagcacactgagtcaaatgggactttccactgggttttgcccaagtacattgggtcaatgggaggtgagccaatgggaaaaacccattgctgccaagtacactgactcaatagggactttccaatgggtttttccattgttggcaagcatataaggtcaatgtgggtgagtcaatagggactttccattgtattctgcccagtacataaggtcaatagggggtgaatcaacaggaaagtcccattggagccaagtacactgcgtcaatagggactttccattgggttttgcccagtacataaggtcaataggggatgagtcaatgggaaaaacccattggagccaagtacactgactcaatagggactttccattgggttttgcccagtacataaggtcaatagggggtgagtcaacaggaaagttccattggagccaagtacattgagtcaatagggactttccaatgggttttgcccagtacataaggtcaatgggaggtaagccaatgggtttttcccattactggcacgtatactgagtcattagggactttccaatgggttttgcccagtacataaggtcaataggggtgaatcaacaggaaagtcccattggagccaagtacactgagtcaatagggactttccattgggttttgcccagtacaaaaggtcaatagggggtgagtcaatgggtttttcccattattggcacgtacataaggtcaataggggtgagtcattgggtttttccagccaatttaattaaaacgccatgtactttcccaccattgacgtcaatgggctattgaaactaatgcaacgtgacctttaaacggtactttcccatagctgattaatgggaaagtaccgttctcgagccaatacacgtcaatgggaagtgaaagggcagccaaaacgtaacaccgccccggttttcccctggaaattccatattggcacgcattctattggctgagctgcgttctacgtgggtataagaggcgcgaccagcgtcggtaccgtcgcagtcttcggtctgaccaccgtagaacgcagagctcctcgctgcaggcggccgcatgggctctaaaccttctaccaggatcccagcacctctgatgctgatcacccggattatgctgatattggactgtatccgtccgacaagctctcttgacggcaggcctcttgcagctgcaggaattgtagtaacaggagataaggcagtcaatgtatatacctcgtctcagacagggtcaatcatagtcaagttgctcccgaatatgcccaaggataaggaggcgtgtgcgaaagacccattagaggcatataacagaacactgactactttgctcactcctcttggcgaatccatccgcaagatccaagggtctgtgtccacgtctggaggaggcaagcaaggccgcctgataggtgctgttattggtagtgtagctcttggggttgcaacagcggcacaaataacagcagctgcggccctaatacaagccaaccagaatgctgccaacatccttcggcttaaggagagcattgctgcaaccaatgaagctgtgcatgaagtcaccgacggattatcacaactatcagtggcagttgggaagatgcagcagtttgtcaatgaccagtttaataatacagcgcgagaattggactgtataaaaatcacacaacaggttggtgtagaactcaacctatacctaactgaattgactacagtattcgggccacagatcacctcccctgcattaactcagctgaccatccaggcactttataatttagctggtggcaatatggattacttattaactaagttaggtatagggaacaatcaactcagctcattaattggcagcggcctgatcactggttaccctatattgtatgactcacagactcaactcttgggcatacaagtgaatttgccctcagtcgggaacttaaataatatgcgtgccacctatttagagaccttatctgtaagtacagccaaaggatatgcctcagcacttgttccaaaagtagtgacacaagtcggttctgtgatagaagagcttgacacctcatactgtatagagtccgatctggatttatattgtactagaatagtgacattccccatgtccccaggtatttattcctgtttaagcggcaacacatcagcttgcatgtattcaaagactgaaggcgcactcactacgccgtatatggcccttaaaggctcagttattgccaattgtaagataacaacatgtagatgtacagaccctcctggtatcatatcgcaaaattatggagaagctgtatccctgatagatagacattcgtgcaatgtcttatcattagacgggataactctgaggctcagtggagaatttgatgcaacttatcaaaagaacatctcaatactagattctcaagtcatcgtgacaggcaatcttgatatatcaactgaacttggaaacgtcaacaattcaatcagcaatgccttggataagttggcaaaaagcaacagcaagctagaaaaagtcaatgtcagactaaccagcacatccgctctcattacctatattgttctgactgtcatttctctagttttcggtgcactaagtctgggtttaacatgttacctgatgtacaaacaaaaggcacaacaaaagaccttgctatggcttgggaataataccctcgatcagatgagagccactacaagagcatgagcggccgcggggatccagacatgataagatacattgatgagtttggacaaaccacaactagaatgcagtgaaaaaaatgctttatttgtgaaatttgtgatgctattgctttatttgtaaccattataagctgcaataaacaagttaacaacaacaattgcattgattttatgtttcaggttcagggggaggtgtgggaggttttttcggatcctctagagtcgacaattattttatttaataacatatagcccaaagacctctatgaacatttagtttcccgtatactcaacggcgcgtgtacacacgcatctctttgcatagcgatgaagtttgttcggcagcagaaaatgcagatatccaacaatctggagaaaacttatcatcacagtggcagtggaaacataccccctctatattcatggtataattatcgtctacagcgtccaggatagtggcgtgagaaaatggagatctgcagccctcctttccatggcatgccgctttattgttcattaaacgcacaatggtctcaacgccagatatgggcatagattctgaagaacccgttgacaatccgaagaagaaggcgtgcaggtctttggaagactcgcacgttggtcttataatgtatgatcgagatgtcaccctaatgccacatggtacaggcttatcgcggtcatggcgatcggacttgtaatttgcaacgatgggcaaaggatcgacgacatgccaaacattctgaacccgtagagatgttaacgatgacgaggatgaatatcccatgctcgctgccatagtatcaagtacaccgcgaataaggacgcgtccaacatcgttatatgcacacaatgggctacacgtgactaacacccccgaatattagtcatatgtgagtttcagtctggctcccatatagcctgtagactatttgtggtttaagtgtgaacgaggcgctgtgaacgagactcgggccgattgtaagaacaagcaaatgcactttccatttaacaagaagtgtagagagaatactcaacctctttggatgtatcctcgag

SEQ ID NO: 30 - DNA, 5381 bp, artificial sequence
  partial plasmid pCD046+Texas NDV-F sequence for HVT113
gagctcagggtatgatactcagctgttattgtggccgaccaggaggactccaatgcttagcattcataagaacgctagagatgctatttaacgatgtgctgtcgtctaaagaatttgtgcatttagcctttaaatgtaaaaccaatgacgcattcactacgctcgtgcgtgcaatttctgggccagggtatgcatattccataacagaaatcgacacttgagaagaggatctgactgtttgggataaaggtcgtttgggtctgtcctagcgatataatttatatgacgatatacattaaacatctgtgtgcagtacttaggtatttaatcatgtcgatgaaatgttatgtgtaaatatcggacaatatagataacgggcacgctgctattgtaacgtgcgcccgcgcgctagtgctgactaatagtgtggatgatgtatacagtatattacaaacggaaatgatacgtaataaattatgtactcttattgatttataaaaacatacatgcagtgttgctatgtcacataattagcctcgcccgtctacgctccactgaagataatgggctcccgctgttcaaaaaaatcagcgtgcgtcgataagactttggtgcagtctcttcggggtcgcaatttagatttgccgcatggagggtatctggggatttttgccaatgctggagcgacgactgtacgattcgtcccatcgggatctagcagaccaatgatgttgacacacatcggccatgcatgtacggacggtctattgcgcgagtttgttattttcgaaggacaagatggaagtgtatatggaaccgacaataatgttagtttgcatttcttagggcggaatctacatgatatcttatccaagcggggtatgagccagagagatgtgatggtcataaagggtaaattttttagatctgaaataacgcagttgcccaaacaacgatcgcgattaaaagaaaaatcggatggttcaattaggacatgcatggattctgtgcgcataaaccataaccgcagcactgttgggcacttcggtaactcaaatgcgaagcgttgcacgtctgcgataactacgcctactatgcacattgttactcctgcatcttaaaaatatatcctgtagtaattttcacagcaatgtcataacatcatctcgctaaagaatgacctgggattggagaagtaatgaatatttgcaaccaatgcattgaataaactaacattaaacgaattcaatagtggatcccccaactccgcccgttttatgactagaaccaatagtttttaatgccaaatgcactgaaatcccctaatttgcaaagccaaacgccccctatgtgagtaatacggggactttttacccaatttcccacgcggaaagccccctaatacactcatatggcatatgaatcagcacggtcatgcactctaatggcggcccatagggactttccacatagggggcgttcaccatttcccagcataggggtggtgactcaatggcctttacccaagtacattgggtcaatgggaggtaagccaatgggtttttcccattactggcaagcacactgagtcaaatgggactttccactgggttttgcccaagtacattgggtcaatgggaggtgagccaatgggaaaaacccattgctgccaagtacactgactcaatagggactttccaatgggtttttccattgttggcaagcatataaggtcaatgtgggtgagtcaatagggactttccattgtattctgcccagtacataaggtcaatagggggtgaatcaacaggaaagtcccattggagccaagtacactgcgtcaatagggactttccattgggttttgcccagtacataaggtcaataggggatgagtcaatgggaaaaacccattggagccaagtacactgactcaatagggactttccattgggttttgcccagtacataaggtcaatagggggtgagtcaacaggaaagttccattggagccaagtacattgagtcaatagggactttccaatgggttttgcccagtacataaggtcaatgggaggtaagccaatgggtttttcccattactggcacgtatactgagtcattagggactttccaatgggttttgcccagtacataaggtcaataggggtgaatcaacaggaaagtcccattggagccaagtacactgagtcaatagggactttccattgggttttgcccagtacaaaaggtcaatagggggtgagtcaatgggtttttcccattattggcacgtacataaggtcaataggggtgagtcattgggtttttccagccaatttaattaaaacgccatgtactttcccaccattgacgtcaatgggctattgaaactaatgcaacgtgacctttaaacggtactttcccatagctgattaatgggaaagtaccgttctcgagccaatacacgtcaatgggaagtgaaagggcagccaaaacgtaacaccgccccggttttcccctggaaattccatattggcacgcattctattggctgagctgcgttctacgtgggtataagaggcgcgaccagcgtcggtaccgtcgcagtcttcggtctgaccaccgtagaacgcagagctcctcgctgcaggcggccgcatgggctccagatcttctaccaggatcccggtacctctaatgctgatcatccgaaccgcgctgacactgagctgtatccgtctgacaagctctcttgatggcaggcctcttgcggctgcagggatcgtggtaacaggagataaagcagtcaacatatacacctcatcccagacagggtcaatcatagttaagttactcccgaatatgcccaaggacaaagaggtgtgtgcaaaagccccattggaggcatacaacaggacactgactactttactcaccccccttggtgattctatccgcaggatacaagagtctgtgactacttccggaggaggcaagcaaggccgcctgataggtgccattatcggcagtgtagctcttggggttgcgacagctgcacagataacagcagcttcggccctgatacaagccaaccagaatgctgccaacatcctccggcttaaagagagcattgctgcaaccaatgaagctgtgcacgaggtcactgacggattatcacaactagcagtggcagtagggaagatgcaacagtttgtcaatgaccagttcaataatacagcgcaagaattggactgtataaaaattgcacagcaggtcggtgtagaactcaacttgtacctaactgaattgactacagtatttgggccacaaatcacttcccctgccttaactcagctgactatccaagcgctttacaatctagctggtggtaatatggattacttgctgactaagttaggtgtagggaacaaccaactcagctcattaattggtagcggcttgatcaccggcaaccctattctgtacgactcacagactcagatcttgggtatacaggtaactttgccttcagttgggaacctgaataatatgcgtgccacctacctggagaccttatctgtaagcacaaccaagggatttgcctcagcacttgtcccaaaagtggtgacacaggtcggttccgtgatagaagaacttgacacctcatactgtatagggaccgacttggatttatactgtacaagaatagtgacattccctatgtctcctggtatttattcttgtctgagcggtaatacatcggcttgcatgtattcaaagactgaaggcgcacttactacgccatatatggctctcaaaggctcagttattgccaattgcaagctgacaacatgtagatgtgcagatcccccaggtatcatatcgcaaaattatggagaagctgtgtccttaatagataggcactcatgcaacgtcttatccttagacgggataactctgaggctcagtggggaatttgatgcaacctatcaaaagaatatctctatactagattctcaagttatagtgacaggcaatcttgatatatcaactgagcttgggaatgtcaacaactcaataagtaatgccctgaataagttagaggaaagcaacagcaaactagacaaagtcaatgtcaaactgaccagcacatctgctctcattacctacatcgttttaactgtcatatctcttgtttttggtgtacttagcctggttctagcatgctacctgatgtacaagcaaaaggcacaacaaaagaccttgttatggcttgggaataatacccttgatcagatgagagccactacaaaaatatgagcggccgcggggatccagacatgataagatacattgatgagtttggacaaaccacaactagaatgcagtgaaaaaaatgctttatttgtgaaatttgtgatgctattgctttatttgtaaccattataagctgcaataaacaagttaacaacaacaattgcattgattttatgtttcaggttcagggggaggtgtgggaggttttttcggatcctctagagtcgacaattattttatttaataacatatagcccaaagacctctatgaacatttagtttcccgtatactcaacggcgcgtgtacacacgcatctctttgcatagcgatgaagtttgttcggcagcagaaaatgcagatatccaacaatctggagaaaacttatcatcacagtggcagtggaaacataccccctctatattcatggtataattatcgtctacagcgtccaggatagtggcgtgagaaaatggagatctgcagccctcctttccatggcatgccgctttattgttcattaaacgcacaatggtctcaacgccagatatgggcatagattctgaagaacccgttgacaatccgaagaagaaggcgtgcaggtctttggaagactcgcacgttggtcttataatgtatgatcgagatgtcaccctaatgccacatggtacaggcttatcgcggtcatggcgatcggacttgtaatttgcaacgatgggcaaaggatcgacgacatgccaaacattctgaacccgtagagatgttaacgatgacgaggatgaatatcccatgctcgctgccatagtatcaagtacaccgcgaataaggacgcgtccaacatcgttatatgcacacaatgggctacacgtgactaacacccccgaatattagtcatatgtgagtttcagtctggctcccatatagcctgtagactatttgtggtttaagtgtgaacgaggcgctgtgaacgagactcgggccgattgtaagaacaagcaaatgcactttccatttaacaagaagtgtagagagaatactcaacctctttggatgtatcctcgag

SEQ ID NO: 31 - DNA, 4600 bp, artificial sequence
  partial plasmid pHM119 sequence for vHVT039
gagctcagggtatgatactcagctgttattgtggccgaccaggaggactccaatgcttagcattcataagaacgctagagatgctatttaacgatgtgctgtcgtctaaagaatttgtgcatttagcctttaaatgtaaaaccaatgacgcattcactacgctcgtgcgtgcaatttctgggccagggtatgcatattccataacagaaatcgacacttgagaagaggatctgactgtttgggataaaggtcgtttgggtctgtcctagcgatataatttatatgacgatatacattaaacatctgtgtgcagtacttaggtatttaatcatgtcgatgaaatgttatgtgtaaatatcggacaatatagataacgggcacgctgctattgtaacgtgcgcccgcgcgctagtgctgactaatagtgtggatgatgtatacagtatattacaaacggaaatgatacgtaataaattatgtactcttattgatttataaaaacatacatgcagtgttgctatgtcacataattagcctcgcccgtctacgctccactgaagataatgggctcccgctgttcaaaaaaatcagcgtgcgtcgataagactttggtgcagtctcttcggggtcgcaatttagatttgccgcatggagggtatctggggatttttgccaatgctggagcgacgactgtacgattcgtcccatcgggatctagcagaccaatgatgttgacacacatcggccatgcatgtacggacggtctattgcgcgagtttgttattttcgaaggacaagatggaagtgtatatggaaccgacaataatgttagtttgcatttcttagggcggaatctacatgatatcttatccaagcggggtatgagccagagagatgtgatggtcataaagggtaaattttttagatctgaaataacgcagttgcccaaacaacgatcgcgattaaaagaaaaatcggatggttcaattaggacatgcatggattctgtgcgcataaaccataaccgcagcactgttgggcacttcggtaactcaaatgcgaagcgttgcacgtctgcgataactacgcctactatgcacattgttactcctgcatcttaaaaatatatcctgtagtaattttcacagcaatgtcataacatcatctcgctaaagaatgacctgggattggagaagtaatgaatatttgcaaccaatgcattgaataaactaacattaaacgaattccgatgtttagtcacgatagacatcggttcgcccagccgtcgaatacagcattatattttagtgttgaaaatgtagggctgcttcctcacttaaaggaggaaatggctcgattcatgtttcatagcagtagaaaaacagattggaccgtcagtaagtttagagggttttatgactttagcactatagataatgtaactgcggcccatcgcatggcttggaaatatatcaaagaactgatttttgcaacagctttattttcttctgtatttaaatgtggcgaattgcacatctgtcgtgccgacagtttgcagatcaacagcaatggagactatgtatggaaaaatggaatatatataacatatgaaaccgaatatccacttataatgattctggggtcagaatcaagcacttcagaaacgcaaaatatgactgcaattattgatacagatgttttttcgttgctttattctattttgcagtatatggcccccgttacggcagatcaggtgcgagtagaacagattaccaacagccacgcccccatctgacccgtccaatattcttgtgtccctgcattttatctcacacaatttatgaacagcatcattaagatcatctcactgcggccgcaagatgggctccagatcttctaccaggatcccggtacctctaatgctgatcatccgaaccgcgctgacactgagctgtatccgtctgacaagctctcttgatggcaggcctcttgcggctgcagggatcgtggtaacaggagataaagcagtcaacatatacacctcatcccagacagggtcaatcatagttaagttactcccgaatatgcccaaggacaaagaggtgtgtgcaaaagccccattggaggcatacaacaggacactgactactttactcaccccccttggtgattctatccgcaggatacaagagtctgtgactacttccggaggaaggagacagagacgctttataggtgccattatcggcagtgtagctcttggggttgcgacagctgcacagataacagcagcttcggccctgatacaagccaaccagaatgctgccaacatcctccggcttaaagagagcattgctgcaaccaatgaagctgtgcacgaggtcactgacggattatcacaactagcagtggcagtagggaagatgcaacagtttgtcaatgaccagttcaataatacagcgcaagaattggactgtataaaaattgcacagcaggtcggtgtagaactcaacttgtacctaactgaattgactacagtatttgggccacaaatcacttcccctgccttaactcagctgactatccaagcgctttacaatctagctggtggtaatatggattacttgctgactaagttaggtgtagggaacaaccaactcagctcattaattggtagcggcttgatcaccggcaaccctattctgtacgactcacagactcagatcttgggtatacaggtaactttgccttcagttgggaacctgaataatatgcgtgccacctacctggagaccttatctgtaagcacaaccaagggatttgcctcagcacttgtcccaaaagtggtgacacaggtcggttccgtgatagaagaacttgacacctcatactgtatagggaccgacttggatttatactgtacaagaatagtgacattccctatgtctcctggtatttattcttgtctgagcggtaatacatcggcttgcatgtattcaaagactgaaggcgcacttactacgccatatatggctctcaaaggctcagttattgccaattgcaagctgacaacatgtagatgtgcagatcccccaggtatcatatcgcaaaattatggagaagctgtgtccttaatagataggcactcatgcaacgtcttatccttagacgggataactctgaggctcagtggggaatttgatgcaacctatcaaaagaatatctctatactagattctcaagttatagtgacaggcaatcttgatatatcaactgagcttgggaatgtcaacaactcaataagtaatgccctgaataagttagaggaaagcaacagcaaactagacaaagtcaatgtcaaactgaccagcacatctgctctcattacctacatcgttttaactgtcatatctcttgtttttggtgtacttagcctggttctagcatgctacctgatgtacaagcaaaaggcacaacaaaagaccttgttatggcttgggaataatacccttgatcagatgagagccactacaaaaatatgagcggccgcggggatccagacatgataagatacattgatgagtttggacaaaccacaactagaatgcagtgaaaaaaatgctttatttgtgaaatttgtgatgctattgctttatttgtaaccattataagctgcaataaacaagttaacaacaacaattgcattcattttatgtttcaggttcagggggaggtgtgggaggttttttcggatcctctagagtcgacaattattttatttaataacatatagcccaaagacctctatgaacatttagtttcccgtatactcaacggcgcgtgtacacacgcatctctttgcatagcgatgaagtttgttcggcagcagaaaatgcagatatccaacaatctggagaaaacttatcatcacagtggcagtggaaacataccccctctatattcatggtataattatcgtctacagcgtccaggatagtggcgtgagaaaatggagatctgcagccctcctttccatggcatgccgctttattgttcattaaacgcacaatggtctcaacgccagatatgggcatagattctgaagaacccgttgacaatccgaagaagaaggcgtgcaggtctttggaagactcgcacgttggtcttataatgtatgatcgagatgtcaccctaatgccacatggtacaggcttatcgcggtcatggcgatcggacttgtaatttgcaacgatgggcaaaggatcgacgacatgccaaacattctgaacccgtagagatgttaacgatgacgaggatgaatatcccatgctcgctgccatagtatcaagtacaccgcgaataaggacgcgtccaacatcgttatatgcacacaatgggctacacgtgactaacacccccgaatattagtcatatgtgagtttcagtctggctcccatatagcctgtagactatttgtggtttaagtgtgaacgaggcgctgtgaacgagactcgggccgattgtaagaacaagcaaatgcactttccatttaacaagaagtgtagagagaatactcaacctctttggatgtatcctcgag

SEQ ID NO: 32 - DNA, 1662 bp, artificial sequence
  NDV Texas F gene (wild type non-modified)
atgggctccagatcttctaccaggatcccggtacctctaatgctgatcatccgaaccgcgctgacactgagctgtatccgtctgacaagctctcttgatggcaggcctcttgcggctgcagggatcgtggtaacaggagataaagcagtcaacatatacacctcatcccagacagggtcaatcatagttaagttactcccgaatatgcccaaggacaaagaggtgtgtgcaaaagccccattggaggcatacaacaggacactgactactttactcaccccccttggtgattctatccgcaggatacaagagtctgtgactacttccggaggaaggagacagagacgctttataggtgccattatcggcagtgtagctcttggggttgcgacagctgcacagataacagcagcttcggccctgatacaagccaaccagaatgctgccaacatcctccggcttaaagagagcattgctgcaaccaatgaagctgtgcacgaggtcactgacggattatcacaactagcagtggcagtagggaagatgcaacagtttgtcaatgaccagttcaataatacagcgcaagaattggactgtataaaaattgcacagcaggtcggtgtagaactcaacttgtacctaactgaattgactacagtatttgggccacaaatcacttcccctgccttaactcagctgactatccaagcgctttacaatctagctggtggtaatatggattacttgctgactaagttaggtgtagggaacaaccaactcagctcattaattggtagcggcttgatcaccggcaaccctattctgtacgactcacagactcagatcttgggtatacaggtaactttgccttcagttgggaacctgaataatatgcgtgccacctacctggagaccttatctgtaagcacaaccaagggatttgcctcagcacttgtcccaaaagtggtgacacaggtcggttccgtgatagaagaacttgacacctcatactgtatagggaccgacttggatttatactgtacaagaatagtgacattccctatgtctcctggtatttattcttgtctgagcggtaatacatcggcttgcatgtattcaaagactgaaggcgcacttactacgccatatatggctctcaaaggctcagttattgccaattgcaagctgacaacatgtagatgtgcagatcccccaggtatcatatcgcaaaattatggagaagctgtgtccttaatagataggcactcatgcaacgtcttatccttagacgggataactctgaggctcagtggggaatttgatgcaacctatcaaaagaatatctctatactagattctcaagttatagtgacaggcaatcttgatatatcaactgagcttgggaatgtcaacaactcaataagtaatgccctgaataagttagaggaaagcaacagcaaactagacaaagtcaatgtcaaactgaccagcacatctgctctcattacctacatcgttttaactgtcatatctcttgtttttggtgtacttagcctggttctagcatgctacctgatgtacaagcaaaaggcacaacaaaagaccttgttatggcttgggaataatacccttgatcagatgagagccactacaaaaatatga

SEQ ID NO: 33 - protein, 553 aa, artificial sequence
  NDV Texas F protein (wild type non-modified)
MGSRSSTRIPVPLMLIIRTALTLSCIRLTSSLDGRPLAAAGIVVTGDKAVNIYTSSQTGSIIVKLLPNMPKDKEVCAKAPLEAYNRTLTTLLTPLGDSIRRIQESVTTSGGRRQRRFIGAIIGSVALGVATAAQITAASALIQANQNAANILRLKESIAATNEAVHEVTDGLSQLAVAVGKMQQFVNDQFNNTAQELDCIKIAQQVGVELNLYLTELTTVFGPQITSPALTQLTIQALYNLAGGNMDYLLTKLGVGNNQLSSLIGSGLITGNPILYDSQTQILGIQVTLPSVGNLNNMRATYLETLSVSTTKGFASALVPKVVTQVGSVIEELDTSYCIGTDLDLYCTRIVTFPMSPGIYSCLSGNTSACMYSKTEGALTTPYMALKGSVIANCKLTTCRCADPPGIISQNYGEAVSLIDRHSCNVLSLDGITLRLSGEFDATYQKNISILDSQVIVTGNLDISTELGNVNNSISNALNKLEESNSKLDKVNVKLTSTSALITYIVLTVISLVFGVLSLVLACYLMYKQKAQQKTLLWLGNNTLDQMRATTKI

SEQ ID NO: 34 - DNA, 1662 bp, artificial sequence
  NDV-F YZCQ wildtype DNA sequence
atgggctccagatcttctaccaggatcccggtacctctaatgctgatcatccgaaccgcgctgacactgagctgtatccgtctgacaagctctcttgatggcaggcctcttgcggctgcagggatcgtggtaacaggagataaagcagtcaacatatacacctcatcccagacagggtcaatcatagttaagttactcccgaatatgcccaaggacaaagaggtgtgtgcaaaagccccattggaggcatacaacaggacactgactactttactcaccccccttggtgattctatccgcaggatacaagagtctgtgactacttccggaggaggcaagcaaggccgcctgataggtgccattatcggcagtgtagctcttggggttgcgacagctgcacagataacagcagcttcggccctgatacaagccaaccagaatgctgccaacatcctccggcttaaagagagcattgctgcaaccaatgaagctgtgcacgaggtcactgacggattatcacaactagcagtggcagtagggaagatgcaacagtttgtcaatgaccagttcaataatacagcgcaagaattggactgtataaaaattgcacagcaggtcggtgtagaactcaacttgtacctaactgaattgactacagtatttgggccacaaatcacttcccctgccttaactcagctgactatccaagcgctttacaatctagctggtggtaatatggattacttgctgactaagttaggtgtagggaacaaccaactcagctcattaattggtagcggcttgatcaccggcaaccctattctgtacgactcacagactcagatcttgggtatacaggtaactttgccttcagttgggaacctgaataatatgcgtgccacctacctggagaccttatctgtaagcacaaccaagggatttgcctcagcacttgtcccaaaagtggtgacacaggtcggttccgtgatagaagaacttgacacctcatactgtatagggaccgacttggatttatactgtacaagaatagtgacattccctatgtctcctggtatttattcttgtctgagcggtaatacatcggcttgcatgtattcaaagactgaaggcgcacttactacgccatatatggctctcaaaggctcagttattgccaattgcaagctgacaacatgtagatgtgcagatcccccaggtatcatatcgcaaaattatggagaagctgtgtccttaatagataggcactcatgcaacgtcttatccttagacgggataactctgaggctcagtggggaatttgatgcaacctatcaaaagaatatctctatactagattctcaagttatagtgacaggcaatcttgatatatcaactgagcttgggaatgtcaacaactcaataagtaatgccctgaataagttagaggaaagcaacagcaaactagacaaagtcaatgtcaaactgaccagcacatctgctctcattacctacatcgttttaactgtcatatctcttgtttttggtgtacttagcctggttctagcatgctacctgatgtacaagcaaaaggcacaacaaaagaccttgttatggcttgggaataatacccttgatcagatgagagccactacaaaaatatga

SEQ ID NO: 35 - protein, 553 aa, artificial sequence
  NDV-F protein from wildtype YZCQ strain  (Amino Acid Sequence of NDV-F of Texas strain with lentogenic cleavage site sequence)
MGSRSSTRIPVPLMLIIRTALTLSCIRLTSSLDGRPLAAAGIVVTGDKAVNIYTSSQTGSIIVKLLPNMPKDKEVCAKAPLEAYNRTLTTLLTPLGDSIRRIQESVTTSGGGKQGRLIGAIIGSVALGVATAAQITAASALIQANQNAANILRLKESIAATNEAVHEVTDGLSQLAVAVGKMQQFVNDQFNNTAQELDCIKIAQQVGVELNLYLTELTTVFGPQITSPALTQLTIQALYNLAGGNMDYLLTKLGVGNNQLSSLIGSGLITGNPILYDSQTQILGIQVTLPSVGNLNNMRATYLETLSVSTTKGFASALVPKVVTQVGSVIEELDTSYCIGTDLDLYCTRIVTFPMSPGIYSCLSGNTSACMYSKTEGALTTPYMALKGSVIANCKLTTCRCADPPGIISQNYGEAVSLIDRHSCNVLSLDGITLRLSGEFDATYQKNISILDSQVIVTGNLDISTELGNVNNSISNALNKLEESNSKLDKVNVKLTSTSALITYIVLTVISLVFGVLSLVLACYLMYKQKAQQKTLLWLGNNTLDQMRATTKI

SEQ ID NO: 36 - DNA, 1662 bp, artificial sequence
  NDV-F Texas wildtype DNA sequence
atgggctctaaaccttctaccaggatcccagcacctctgatgctgatcacccggattatgctgatattggactgtatccgtccgacaagctctcttgacggcaggcctcttgcagctgcaggaattgtagtaacaggagataaggcagtcaatgtatatacctcgtctcagacagggtcaatcatagtcaagttgctcccgaatatgcccaaggataaggaggcgtgtgcgaaagacccattagaggcatataacagaacactgactactttgctcactcctcttggcgaatccatccgcaagatccaagggtctgtgtccacgtctggaggaggcaagcaaggccgcctgataggtgctgttattggtagtgtagctcttggggttgcaacagcggcacaaataacagcagctgcggccctaatacaagccaaccagaatgctgccaacatccttcggcttaaggagagcattgctgcaaccaatgaagctgtgcatgaagtcaccgacggattatcacaactatcagtggcagttgggaagatgcagcagtttgtcaatgaccagtttaataatacagcgcgagaattggactgtataaaaatcacacaacaggttggtgtagaactcaacctatacctaactgaattgactacagtattcgggccacagatcacctcccctgcattaactcagctgaccatccaggcactttataatttagctggtggcaatatggattacttattaactaagttaggtatagggaacaatcaactcagctcattaattggcagcggcctgatcactggttaccctatattgtatgactcacagactcaactcttgggcatacaagtgaatttgccctcagtcgggaacttaaataatatgcgtgccacctatttagagaccttatctgtaagtacagccaaaggatatgcctcagcacttgttccaaaagtagtgacacaagtcggttctgtgatagaagagcttgacacctcatactgtatagagtccgatctggatttatattgtactagaatagtgacattccccatgtccccaggtatttattcctgtttaagcggcaacacatcagcttgcatgtattcaaagactgaaggcgcactcactacgccgtatatggcccttaaaggctcagttattgccaattgtaagataacaacatgtagatgtacagaccctcctggtatcatatcgcaaaattatggagaagctgtatccctgatagatagacattcgtgcaatgtcttatcattagacgggataactctgaggctcagtggagaatttgatgcaacttatcaaaagaacatctcaatactagattctcaagtcatcgtgacaggcaatcttgatatatcaactgaacttggaaacgtcaacaattcaatcagcaatgccttggataagttggcaaaaagcaacagcaagctagaaaaagtcaatgtcagactaaccagcacatccgctctcattacctatattgttctgactgtcatttctctagttttcggtgcactaagtctgggtttaacatgttacctgatgtacaaacaaaaggcacaacaaaagaccttgctatggcttgggaataataccctcgatcagatgagagccactacaagagcatga

SEQ ID NO: 37 - protein, 553 aa, artificial sequence
  NDV-F protein from wildtype Texas strain (Amino Acid Sequence of NDV-F VIId wt YZCQ with lentogenic cleavage site sequence)
MGSKPSTRIPAPLMLITRIMLILDCIRPTSSLDGRPLAAAGIVVTGDKAVNVYTSSQTGSIIVKLLPNMPKDKEACAKDPLEAYNRTLTTLLTPLGESIRKIQGSVSTSGGGKQGRLIGAVIGSVALGVATAAQITAAAALIQANQNAANILRLKESIAATNEAVHEVTDGLSQLSVAVGKMQQFVNDQFNNTARELDCIKITQQVGVELNLYLTELTTVFGPQITSPALTQLTIQALYNLAGGNMDYLLTKLGIGNNQLSSLIGSGLITGYPILYDSQTQLLGIQVNLPSVGNLNNMRATYLETLSVSTAKGYASALVPKVVTQVGSVIEELDTSYCIESDLDLYCTRIVTFPMSPGIYSCLSGNTSACMYSKTEGALTTPYMALKGSVIANCKITTCRCTDPPGIISQNYGEAVSLIDRHSCNVLSLDGITLRLSGEFDATYQKNISILDSQVIVTGNLDISTELGNVNNSISNALDKLAKSNSKLEKVNVRLTSTSALITYIVLTVISLVFGALSLGLTCYLMYKQKAQQKTLLWLGNNTLDQMRATTRA

SEQ ID NO: 38 - DNA, 622 bp, artificial sequence
  MDV gB promoter
cgatgtttagtcacgatagacatcggttcgcccagccgtcgaatacagcattatattttagtgttgaaaatgtagggctgcttcctcacttaaaggaggaaatggctcgattcatgtttcatagcagtagaaaaacagattggaccgtcagtaagtttagagggttttatgactttagcactatagataatgtaactgcggcccatcgcatggcttggaaatatatcaaagaactgatttttgcaacagctttattttcttctgtatttaaatgtggcgaattgcacatctgtcgtgccgacagtttgcagatcaacagcaatggagactatgtatggaaaaatggaatatatataacatatgaaaccgaatatccacttataatgattctggggtcagaatcaagcacttcagaaacgcaaaatatgactgcaattattgatacagatgttttttcgttgctttattctattttgcagtatatggcccccgttacggcagatcaggtgcgagtagaacagattaccaacagccacgcccccatctgacccgtccaatattcttgtgtccctgcattttatctcacacaatttatgaacagcatcattaagatcatctcact

SEQ ID NO: 39 - DNA, 4850 bp, artificial sequence
  Partial plasmid SORF3-US2 gpVar-Ewtsyn sequence for vHVT202
taaaatgggatctatcattacattcgttaagagtctggataattttactgtttgccagcttcgatcttggaacgtactgtggatagtgccttacttggaatcgtgaaaatttgaaacgtccattatttggatatcttccggttgtcccatatcccgccctggtaccgctcggataccttgcccgtatggattcgtattgacagtcgcgcaatcggggaccaacaacgcgtgggtccacactcattcggaaattttccgatgattctgaatatttattgccgctcgttacgagtcgttggacatatctgtaatacatttcttcttctgaaggatcgctgcacatttgatctatacattggccaggatgttcaagtctcagatgttgcattctggcacagcacaactttatggcatttccgatgtaatcgtccggcagccctgggggagttctatattcgcatattgggatggtaaggacaatagcagatctcgcaacctccagggaggctataataacgtttttaaaggatggatttctcataaaaatctgtcgcaaattacactgagaatatcctttactagcgccgattgagagcatcgtcgtccaattttctaaatggaaagaaaacaaggcgggcaagagtgttccaaacattttcattttcggcgaatctctcaaatcccatggcgtgcaattgattgcaaaattggcacttccgttcacgtttgtatctccaaactctaagacacttttaattgaaaaactacgttctagtgtggaaagaaacctataggcagaccatagaactatttgacaccacatatctttttgtatgtcaaactgaccatgatcgtatgttgctgaatgcactagggcaattcgctcgcgcgactccatacattgaataattccacacgtcagctcatcggttagcaaggtccagtagttgaagtcatttatttttccccgcggctggccaaatctacctctgggaatatccaagttgtcgaatatgatcgcaccggctctggtcatggtgaaggaacttgtagcataaagacgcaggtatcataggggtaatatttttttattcactcacatactaaaagtaacgcatattagcaccatgtatgggctatcaattgacatttgcgtagcactacatcacgattatgtacaacataatgggacaacatatgcctgcaggttagtcatatgttacttggcagaggccgcatggaaagtccctggacgtgggacatctgattaatacgtgaggaggtcagccatgttctttttggcaaaggactacggtcattggacgtttgattggcatgggatagggtcagccagagttaacagtgttcttttggcaaagggatacgtggaaagtcccgggccatttacagtaaactgatacggggacaaagcacagccatatttagtcatgtattgcttggcagagggtctatggaaagtccctggacgtgggacgtctgattaatatgaaagaaggtcagccagaggtagctgtgtcctttttggcaaagggatacggttatgggacgtttgattggactgggatagggtcagccagagttaacagtgttcttttggcaaaggaaacgtggaaagtcccgggccatttacagtaaactgatactgggacaaagtacacccatatttagtcatgttctttttggcaaagagcatctggaaagtcccgggcagcattatagtcacttggcagagggaaagggtcactcagagttaagtacatctttccagggccaatattccagtaaattacacttagttttatgcaaatcagccacaaaggggattttcccggtcaattatgactttttccttagtcatgcggtatccaattactgccaaattggcagtacatactaggtgattcactgacatttggccgtcctctggaaagtccctggaaaccgctcaagtactgtatcatggtgactttgcatttttggagagcacgccccactccaccattggtccacgtaccctatgggggagtggtttatgagtatataaggggctccggtttagaagccgggcagagcggccgcatgacaaacctgcaagatcaaacccaacagattgttccgttcatacggagccttctgatgccaacaaccggaccggcgtccattccggacgacaccctggagaagcacactctcaggtcagagacctcgacctacaatttgactgtgggggacacagggtcagggctaattgtctttttccctggattccctggctcaattgtgggtgctcactacacactgcagagcaatgggaactacaagttcgatcagatgctcctgactgcccagaacctaccggccagctacaactactgcaggctagtgagtcggagtctcacagtaaggtcaagcacactccctggtggcgtttatgcactaaacggcaccataaacgccgtgaccttccaaggaagcctgagtgaactgacagatgttagctacaacgggttgatgtctgcaacagccaacatcaacgacaaaattgggaacgtcctagtaggggaaggggtaaccgtcctcagcttacccacatcatatgatcttgggtatgtgaggcttggtgaccccatacccgctatagggcttgacccaaaaatggtagcaacatgtgacagcagtgacaggcccagagtctacaccataactgcagccgataattaccaattctcatcacagtaccaaacaggtggggtaacaatcacactgttctcagccaacattgatgccatcacaagtctcagcgttgggggagagctcgtgttcaaaacaagcgtccaaagccttgtactgggcgccaccatctaccttataggctttgatgggactgcggtaatcaccagagctgtggccgcaaacaatgggctgacggccggcatcgacaatcttatgccattcaatcttgtgattccaaccaatgagataacccagccaatcacatccatcaaactggagatagtgacctccaaaagtgatggtcaggcaggggaacagatgtcatggtcggcaagtgggagcctagcagtgacgatccatggtggcaactatccaggagccctccgtcccgtcacactagtggcctacgaaagagtggcaacaggatctgtcgttacggtcgctggggtgagcaacttcgagctgatcccaaatcctgaactagcaaagaacctggttacagaatatggccgatttgacccaggagccatgaactacacgaaattgatactgagtgagagggaccgccttggcatcaagaccgtctggccaacaagggagtacactgactttcgtgagtacttcatggaggtggccgacctcaactctcccctgaagattgcaggagcatttggcttcaaagacataatccgggccataaggaggtgagcggccgcgatatcaataaaatatctttattttcattacatctgtgtgttggttttttgtgtgaatcgatagtactaacatacgctctccatcaaaacaaaacgaaacaaaacaaactagcaaaataggctgtccccagtgcaagtgcaggtgccagaacatttctcttctagacctgcaggcccggggcaagtagatgcaatttcctcacactagttgggtttatctactattgaattttcccctatctgtgatacacttgggagcctctacaagcatattgccatcatgtacgtttttatctactgtcttaacgcccatgggaacggaggcgtcgtcgtcatgtattggacggcaacataggcagcaacacaaattgcgtttaggtggggtgcatgtggactcgataccaagcccctgcagctggggaacgtctggtggagagccgataatttgatatacgcacgccatattactgtcgttgaagtacgccttatcttctatgttttcaaatttaggttcccaagtggacgtgagaagtgtttgtatctcacatggaatggcccaaggcattccagcccaggtgcctggtactttaatggcaaacaaacgttttggtagaggtattgattctattgcagttctgcagatatctgcagccccgagtatccacaggctatacgatacgttatcggaggcctccgattctagcattacatagccggtcagtagatcctgccattcggtagcgcaaccggctacatcttcaaacagtctcacaataaatgcatctctcgttcctgccaatccggaaccgggcataccactcccgcctgccgatttaattctcacaattgggcgatgccggcggggcaaaacgaatgtggatttggcaaaccgacacaggtctgctgtacggactaatatgggcacacccacatcattcttcagatgctccatgcattgttctatgagaaagatccatagggtggaggcagcgtcacgagatcgcccaggcaatcgatcgcattcgtctagtaaagtgacgagagttatcatgcacacacccatgcccacgccttccgaataactggagctgtggaagatcggaaacgtctttttgactgccggtctcgtactactttcgcacaggtgtatacccggacgcgtactatatattttatatcatccaacgtcccgaaattacatacgtggcggcgatggaagtagatgttgagtcttcgaaagtaagtgcctcgaatatgggtattgtctgtgaaaatatcgaaagcggtacgacggttgcagaaccgtcgatgtcgccagatactagtaacaatagcttcgataacgaagacttccgtgggcctgaatacgatgtggagata

SEQ ID NO: 40 - DNA, 4943 bp, artificial sequence
  Partial plasmid SB1US2 gpVIIdwtsyn sequence for vSB1-010
tctcgtctaaaacgctccagtgctttacagttcgataatctggacctggggacgcgtataggatcgttcctccacatgcgctgctgtcggtatctcgaatccccggtattcagttgaatcgttggcggagtgtcctcctggactctgcaatgttccctagccgtcttcactatctcgtgcaaggctctataatacagttcctctgcagacccgtcgttgctcttcccttctgcgtcgttagttatttctgtaggctccagacgatttgcctgcatttgtgcgcaacataatctgattgcattccctatctcgtcttccggtaatcccataggtgttcggtattcgcagataggtagagaaagcaccactgcaaatcgtgcaatttccattgccccaaccaatattttttttaagaacggcatcgccgttaatgtacctcgggcattgtgacgatcgaaacccttatggatgcctaaagagagcattgcggtccagttctccaggtgaaaagagaatagcgcgggtagaaacgggccgattagttttatcttcgccgcgtccctaatatcccaagttctgcagtataacttccatcgtccgttttcgacaaggtccggcgcgacatagtttgaaatgtcatctatcagaaacatctcgcccatcgtagaaaaaaacctgtacgcagaccataaaaccattcggtaccacatatccttgtgtatatcaaacgatatgttggttatgtcgttggcggatgttgtatgaaatagagctaagcgttctctggattccacgcactgaacgattccgttagtcaattcatctgctaacataggccaaaagtttattcgtgttacttttctcggcggtttggcaaaacgcccccttggcacatccatgtcattaaatacagcggcataactcctactcatgtgttccatagcccaggtttctgttcggtctgctactacgatcagatcagtggcgcgatcagatgcgtgggatgaatgaagtgtatccgaaagcagttttgagatatacgctaaactgtacgacgattgtggcactaaacgaagctttgcgcgacccccatcccacgccctgcaggttagtcatatgttacttggcagaggccgcatggaaagtccctggacgtgggacatctgattaatacgtgaggaggtcagccatgttctttttggcaaaggactacggtcattggacgtttgattggcatgggatagggtcagccagagttaacagtgttcttttggcaaagggatacgtggaaagtcccgggccatttacagtaaactgatacggggacaaagcacagccatatttagtcatgtattgcttggcagagggtctatggaaagtccctggacgtgggacgtctgattaatatgaaagaaggtcagccagaggtagctgtgtcctttttggcaaagggatacggttatgggacgtttgattggactgggatagggtcagccagagttaacagtgttcttttggcaaaggaaacgtggaaagtcccgggccatttacagtaaactgatactgggacaaagtacacccatatttagtcatgttctttttggcaaagagcatctggaaagtcccgggcagcattatagtcacttggcagagggaaagggtcactcagagttaagtacatctttccagggccaatattccagtaaattacacttagttttatgcaaatcagccacaaaggggattttcccggtcaattatgactttttccttagtcatgcggtatccaattactgccaaattggcagtacatactaggtgattcactgacatttggccgtcctctggaaagtccctggaaaccgctcaagtactgtatcatggtgactttgcatttttggagagcacgccccactccaccattggtccacgtaccctatgggggagtggtttatgagtatataaggggctccggtttagaagccgggcagagcggccgcatgggctccaaaccttctaccaggatcccagcacctctgatgctgatcacccggattatgctgatattgggctgtatccgtccgacaagctctcttgacggcaggcctcttgcagctgcaggaattgtagtaacaggagataaggcagtcaatgtatacacttcgtctcagacagggtcaatcatagtcaagttgctcccgaatatgcccagggataaggaggcgtgtgcaaaagccccattagaggcatataacagaacactgactactttgctcactcctcttggcgactccatccgcaagatccaagggtctgtgtccacatctggaggaggcaagcaaggccgcctgataggtgctgttattggcagtgtagctcttggggttgcaacagcggcacagataacagcagctgcggccctaatacaagccaaccagaatgccgccaacatcctccggcttaaggagagcattgctgcaaccaatgaagctgtgcatgaagtcaccgacggattatcacaactatcagtggcagttgggaagatgcagcagtttgtcaatgaccagtttaataatacggcgcgagaattggactgtataaaaatcacacaacaggttggtgtagaactcaacctatacctaactgaattgactacagtattcgggccacagatcacctcccctgcattaactcagctgaccatccaggcactttataatttagctggtggcaatatggattacttattaactaagttaggtatagggaacaatcaactcagctcgttaattggtagcggcctgatcactggttaccctatactgtatgactcacagactcaactcttgggcatacaagtgaatttaccctcagtcgggaacttaaataatatgcgtgccacctatttggagaccttatctgtaagtacaaccaaaggatatgcctcagcacttgtcccgaaagtagtgacacaagtcggttccgtgatagaagagcttgacacctcatactgtatagagtccgatctggatttatattgtactagaatagtgacattccccatgtccccaggtatttattcctgtttgagcggcaacacatcagcttgcatgtattcaaagactgaaggcgcactcactacgccgtatatggcccttaaaggctcagttattgccaattgtaaaataacaacatgtagatgtacagaccctcctggtatcatatcgcaaaattatggagaagctgtatccctgatagatagacattcgtgcaatgtcttatcattagacgggataactctaaggctcagtggggaatttgatgcaacttatcaaaagaacatctcaatactagattctcaagtcatcgtgacaggcaatcttgatatatcaactgaacttggaaacgtcaacaattcaatcagcaatgccttggataggttggcagaaagcaacagcaagctagaaaaagtcaatgtcagactaaccagcacatctgctctcattacctatattgttctaactgtcatttctctagttttcggtgcacttagtctggtgttagcgtgttacctgatgtacaaacagaaggcacaacaaaagaccttgctatggcttgggaataataccctcgatcagatgagagccactacaagagcatgagcggccgcgatatcaataaaatatctttattttcattacatctgtgtgttggttttttgtgtgaatcgatagtactaacatacgctctccatcaaaacaaaacgaaacaaaacaaactagcaaaataggctgtccccagtgcaagtgcaggtgccagaacatttctcttctagacctgcaggggagtctgtgcaaggttaatgaccctcgcagttcattcggaagttataactgccgccttcgcacatttctttttgtcctgttttgtattgccataacagataggaattgaaacctgatcctcctgttttttgcagcatggccagcaacagaatactttgtcggatcgactacttgcgcgagatggttccgttcttggaggtttcggcgggtcgggtggagaacctattattttatacacacacgtcataccgttgtcgcgaaaatgttctttgtcttctgccgtctcgaacgtcggttcccacgtagacgttaggagcgttggaatggtatcaggaagagcccacggcatgccggaccaagtacccgctactttgaccgcgagcagtctcttcggtaatgggatgtattccagagcagcgcggcagagatcagcggcccccactatccacagactgtatgaagtgttttctgaaacatcggactccaacatcaaatatccagacataacatcttgccattcggaagcacatccgccgacatcttcaaatagcctaactataaacgagtctctagttcctgctaacccagtacctcgaatgccagtcccatccggtgggttcgtcctgataatcggtctctgacgccgaggaagaactaaaaggggtctggaaaagcggaacagatctgcagaccgaacgactacagacacgcccacatcatcatgtatctgttccatgcattgctttatgagaaaaatccataaggccgaggcggcatctctagatctcccggggagtctctcgcactcatctaggagagtgacgacagttatcatagacacgcccatttgtgcaccaaacgaaaagttcctgtactggtggagcgtcggcgcgggaatcggtccgtgctctgaaaccagtgtctagacagaagaccatccggtaaattctggtgtatgaactgacggtctccagacgaacgtcgaagacattaacgatggaaactaacgagctttcttcaaaagtgtctgattacaacgctaatagaccttacgaaactatacgcagcgataccagtgacacagatccgtcggtgtcg

SEQ ID NO: 41 - DNA, 1362 bp, artificial sequence
  IBDV DNA encoding VP2 protein of IBDV E strain
atgacaaacctgcaagatcaaacccaacagattgttccgttcatacggagccttctgatgccaacaaccggaccggcgtccattccggacgacaccctggagaagcacactctcaggtcagagacctcgacctacaatttgactgtgggggacacagggtcagggctaattgtctttttccctggattccctggctcaattgtgggtgctcactacacactgcagagcaatgggaactacaagttcgatcagatgctcctgactgcccagaacctaccggccagctacaactactgcaggctagtgagtcggagtctcacagtaaggtcaagcacactccctggtggcgtttatgcactaaacggcaccataaacgccgtgaccttccaaggaagcctgagtgaactgacagatgttagctacaacgggttgatgtctgcaacagccaacatcaacgacaaaattgggaacgtcctagtaggggaaggggtaaccgtcctcagcttacccacatcatatgatcttgggtatgtgaggcttggtgaccccatacccgctatagggcttgacccaaaaatggtagcaacatgtgacagcagtgacaggcccagagtctacaccataactgcagccgataattaccaattctcatcacagtaccaaacaggtggggtaacaatcacactgttctcagccaacattgatgccatcacaagtctcagcgttgggggagagctcgtgttcaaaacaagcgtccaaagccttgtactgggcgccaccatctaccttataggctttgatgggactgcggtaatcaccagagctgtggccgcaaacaatgggctgacggccggcatcgacaatcttatgccattcaatcttgtgattccaaccaatgagataacccagccaatcacatccatcaaactggagatagtgacctccaaaagtgatggtcaggcaggggaacagatgtcatggtcggcaagtgggagcctagcagtgacgatccatggtggcaactatccaggagccctccgtcccgtcacactagtggcctacgaaagagtggcaacaggatctgtcgttacggtcgctggggtgagcaacttcgagctgatcccaaatcctgaactagcaaagaacctggttacagaatatggccgatttgacccaggagccatgaactacacgaaattgatactgagtgagagggaccgccttggcatcaagaccgtctggccaacaagggagtacactgactttcgtgagtacttcatggaggtggccgacctcaactctcccctgaagattgcaggagcatttggcttcaaagacataatccgggccataaggaggtga

SEQ ID NO: 42 - protein, 453 aa, artificial sequence
  IBDV VP2 protein of IBDV E strain
MTNLQDQTQQIVPFIRSLLMPTTGPASIPDDTLEKHTLRSETSTYNLTVGDTGSGLIVFFPGFPGSIVGAHYTLQSNGNYKFDQMLLTAQNLPASYNYCRLVSRSLTVRSSTLPGGVYALNGTINAVTFQGSLSELTDVSYNGLMSATANINDKIGNVLVGEGVTVLSLPTSYDLGYVRLGDPIPAIGLDPKMVATCDSSDRPRVYTITAADNYQFSSQYQTGGVTITLFSANIDAITSLSVGGELVFKTSVQSLVLGATIYLIGFDGTAVITRAVAANNGLTAGIDNLMPFNLVIPTNEITQPITSIKLEIVTSKSDGQAGEQMSWSASGSLAVTIHGGNYPGALRPVTLVAYERVATGSVVTVAGVSNFELIPNPELAKNLVTEYGRFDPGAMNYTKLILSERDRLGIKTVWPTREYTDFREYFMEVADLNSPLKIAGAFGFKDIIRAIRR

SEQ ID NO: 43 - DNA, 884 bp, artificial sequence
  Guinea pig CMV promoter
ttagtcatatgttacttggcagaggccgcatggaaagtccctggacgtgggacatctgattaatacgtgaggaggtcagccatgttctttttggcaaaggactacggtcattggacgtttgattggcatgggatagggtcagccagagttaacagtgttcttttggcaaagggatacgtggaaagtcccgggccatttacagtaaactgatacggggacaaagcacagccatatttagtcatgtattgcttggcagagggtctatggaaagtccctggacgtgggacgtctgattaatatgaaagaaggtcagccagaggtagctgtgtcctttttggcaaagggatacggttatgggacgtttgattggactgggatagggtcagccagagttaacagtgttcttttggcaaaggaaacgtggaaagtcccgggccatttacagtaaactgatactgggacaaagtacacccatatttagtcatgttctttttggcaaagagcatctggaaagtcccgggcagcattatagtcacttggcagagggaaagggtcactcagagttaagtacatctttccagggccaatattccagtaaattacacttagttttatgcaaatcagccacaaaggggattttcccggtcaattatgactttttccttagtcatgcggtatccaattactgccaaattggcagtacatactaggtgattcactgacatttggccgtcctctggaaagtccctggaaaccgctcaagtactgtatcatggtgactttgcatttttggagagcacgccccactccaccattggtccacgtaccctatgggggagtggtttatgagtatataaggggctccggtttagaagccgggcaga

SEQ ID NO: 44 - DNA, 30 bp, artificial sequence
  primer HM101
ccggaattccgatgtttagtcacgatagac

SEQ ID NO: 45 - DNA, 35 bp, artificial sequence
  Primer HM102
ataagagcggccgcagtgagatgatcttaatgatg

SEQ ID NO: 46 - DNA, 38 bp, artificial sequence
  primer F-ATG
tatagcggccgcaagatgggctccagatcttctaccag

SEQ ID NO: 47 - DNA, 34 bp, artificial sequence
  Primer F-STOP
cgaggcggccgctcatatttttgtagtggctctc